European Patent Specification EP 3 346 011 B1, published May 20, 2026. Title: Adipate (ester or thioester) synthesis. Applicant: Genomatica, Inc. 4757 Nexus Center Drive, San Diego, CA 92121 USA. The sequence listing filed with the application follows.

SEQUENCE LISTING (148 sequences)

SEQ ID NO: 1 - protein, 419 aa, Penicillium chrysogenum
MSNAQQRLSQVSSHFGPGGKKGAAAITEKHPDDIVVTCALRTALTKGGKGGFKDTAGADLLAGVFKAVLNKSGVDPSSVQDIAVGSVLAPGGGATEFRAAALVAGFPESTAVKSLNRQCSSGLQAIADIANAIQSGMIDVGIGAGVESMSSQYGPGAVTEFSDLLESHPESANCKVPMGVLSENMAKDRGVTRASQDSFAAQSYQKAVAAQKAGLFNEEIAPLDVKWTDPKTGEEKTITVKADDGVRQGITAESLGKIKPAFAKDGSIHAGNASQISDGAAAVLLMKRSTAERLGQKILGKYVTASVVGVKPLLMGVGPWKAIPVALEKAGITKDDVDIYEINEAFASQCVWCVNELGIPAEKVNPKGGAIAFGHPLGCTGARQVSTLFTELKRTNKKIGVTSMCVGTGMGMAAVWVSE

SEQ ID NO: 2 - protein, 418 aa, Penicillium chrysogenum
MSSPQQRLNSVANQLAPGSARQKILAKNPDDVVITYLARTPLTKARKGGLKDTTVDDLLISLLTTVREKSNLDPNLVEDVCVGNVLCPGSAYVARSAVLAAGYPVTAAASIANRFCSSGLLAVQNIANQIIAGSIDVGVAVGAESMSKNADGGAPEMSERITKHPIASQNSQPMGQTSENVANQFNISREQHDRFAANSFQKAERAQKAGWLEDEIVPVRTQIKDPKTGEVKDIVVVRDDGIRYGTTPESLGKVRAAFPQWAPSATTGGNASQITDGAAALVLMKRSRAQQLGQPIVAKFCGATVSGLEPRIMGIGPSLAIPKILSKFNLSKDDIDIFEINEAFSSMGVYCVNKLGLDESKVNPRGGAIAFGHPLGATGARQVVTALSELRRQDKRVAVTSMCVGTGMGMAGIFVSEH

SEQ ID NO: 3 - protein, 418 aa, Penicillium chrysogenum
MAADRLSSLLSHLKPGATNGLAAITQKNPDDVVITLAIRTPLTKARKGGFKDTELDYMIYALLKETLAKSQIDPALIEDVCLGNVNEVKAAYMVRAAALAAGIPHTAGASSVNRFCSSGLKAVQDIANQIQLGAIDVGVALGAELMSASGDRLDRPFNEEVLRNQEAADCMQPMGQTSENVGKDFDIPREQQDRYAAESFRRAEAAQNNGWLDDEIAPIAVKVKDPKTGEVKEVTLSRDDGIRPGTTFESLSKIRPAFPQFGDKSTGGNSSQVTDGAASVLLMRRSKAIELNQPILAKFCGATVAGVPPRVMGIGPTAAIPKLLSKFQLDKNDIDIYEINEAFASMAVYCVKNLGLDHAKVNPRGGAIALGHPLGATGARQIATILSEARRTKSKILVTSMCIGTGQGMAGLFVNEQL

SEQ ID NO: 4 - protein, 413 aa, Penicillium chrysogenum
MASPIPRGLRQVLQKSSNDIVILSSLRTPVTRAKKGGFKDAYPEELLASVLQATLKANPNLDPAQIDDVLIGSVLQELGGAKAGRMGQIHAGFPHSVPFNTINRQCSSGLAAITTIANGIRAGAINVGVGGGMESMTRNYGSRAIPTVLWPELKESYSQDARDCIMPMGITSENVASRYGVSRADQDAFAVESHAKASAAQKAGRFDSEIVSVTTKTLDPENPDAPARDVTVSQDDGIRHGLSIEKVGALKPAFSPTGASTAGNSSQVSDGAAATLLMRRSTAEELGLSGSIKARWVASAVAGCAPDEMGVGPAVAIPKLLQTVGVEVPEVGVWEINEAFASQALYSVRKLGIDQAKVNPNGGAIAIGHPLGATGARQLATLLPELERSGQEIGVISMCIGTGMGMAGMFVRE

SEQ ID NO: 5 - protein, 401 aa, Acinetobacter sp.
MLNAYIYDGLRTPFGRHAGELASIRPDDLAGLVIQRLIEKTGVAGADIEDVIFGDTNQAGEDSRNIARHAALLAGLPVTVPGQTVNRLCASGLAAIIDSARAITCGEGDLYIAGGVESMSRAPFVMGKAESAYSRDAKIYDTTIGTRFPNKKIVAQYGGHSMPETGDNVAVEYGISREQADLFAAQSQAKYQKALEEGFFAGEITAVEVSQGKKLPPKQVTEDEHPRPSSTLEALSKLKPLFEGGVVTAGNASGINDGAAALLIGSEVAGQKYGLTPMAKILSAAAAGVEPRIMGAGPIEAIKKAVARAGLTLDDLDIIEINEAFASQVLSCLKGLGIDFNDPRVNPNGGAIAVGHPLGASGARLALTVARELQRRNKKYAVVSLCIGVGQGLAMVIENVS

SEQ ID NO: 6 - protein, 393 aa, Clostridium kluyveri
MREVVIVSAVRTAIGSFGGTLKDVSAVDLGAIVIKEAVKRAGIKPEQVDEVIFGNVIQAGVGQSLARQSAVYAGLPVEVPAFTVNKLCGSGLRTVSLAASLISNGDADTIVVGGSENMSASPYLIPKARFGYRMGEAKIYDAMLHDGLIDSFNNYHMGITAENIAEKWGITREDQDKFALASQQKAEAAIKAGKFKDEIVPVTVKMKKKEVVFDTDEDPRFGTTIETLAKLKPAFKRDGTGTVTAGNSSGINDSSAALILMSADKAKELGVKPMAKYVDFASAGLDPAIMGYGPYYATKKVLAKTNLTIKDFDLIEANEAFAAQSIAVARDLEFDMSKVNVNGGAIALGHPVGCSGARILVTLLHEMQKRDAKKGLATLCIGGGQGTAVVVER

SEQ ID NO: 7 - protein, 391 aa, Clostridium kluyveri
MKDAVIVSAVRTAIGSFGGTLKDISAVDLGAIVIKEAVKRAGIKPEQVDEVIFGNVIQAGLGQSPARQAAVKAGIPVEVPAFTLNKVCGSGLRSVSLAAQLIKIGDDDIVVVGGTENMSAAPYLLPKARWGHRMGEGKLVDAMIKDGLWEAFNNYHMGITAENIAEKWGITRDMQDEFALASQQKAEAAIKAGKFKDEIVPVTVKQKKKEIIFDTDEFPRFGTTIEALAKLKPSFKKDGTVTAGNASGINDAAAALVVMSADKAKELGIKPLAKIVSYGSKGLDPTIMGYGPFYATKLALEKANLSIADLDLIEANEAFASQSLAVAKDLEFDMSKVNVNGGAIALGHPVGCSGARILVTLLYEMQRRDAKKGLATLCIGGGMGTALIVER

SEQ ID NO: 8 - protein, 391 aa, Clostridium kluyveri
MREVVIVSAVRTAIGSFGGTLKDVPAVELGAVVIKEAVKRANVKPEQIDEVIFGNVIQAGLGQSPARQAAVKAGIPVEVPAFTLNKVCGSGLRSVSLAAQVIKAGDADIVVVGGMENMSAAPYVLPKARWGHRMGEGKIVDAMIKDGLWEAFNNYHMGITAENIAEKWGLTREEQDEFSAASQQKAEAAQKAGKFKDEIVPVTVKIKKKEVVFDTDEYIKPGTTVETLAKLRPAFKKDGTVTAGNASGINDAAAALVVMSADKAKELGIKPLAKIVSYGSAGLDPTIMGYGPFHATKAALEKANLSVADLDLIEANEAFASQSLAVAKDLEFDMSKVNVNGGAIALGHPVGASGARILVTLLHEMQRRDAKKGLATLCIGGGMGTALIVER

SEQ ID NO: 9 - protein, 408 aa, Corynebacterium glutamicum
MNPQDIVICSPLRTPVGAYGGSFTGVPVEELATTVINAIVEATGITGDDVDDLILGQASPNGAAPALGRVVALDSKLGQNVPGMQLDRRCGSGLQAIVTAAAHVASGAADLIIAGGAESMSRVEYTVSGDIRWGVKGGDMQLRDRLAEARETAGGRNHPIPGGMIETAENLRREYGISREEQDKISAASQQRWGKAADAGLFDDEIVPVTVPAKKRGQEPTIVSRDEHGRPGTTVEKLAALRPIMGRQDAEATVTAGNASGQNDGAAAVIVTTRAKAEEKGLRPVMRLAGWSVAAVPPETMGIGPVPATKKVLDRLGLTLEDIGAIELNEAFAAQALSVLKEWNISWEDERVNPLGSGISMGHPVGATGARMAVTLAHRMQRENTQYGLATMCIGGGQGLAAVFEKEN

SEQ ID NO: 10 - protein, 401 aa, Escherichia coli
MREAFICDGIRTPIGRYGGALSSVRADDLAAIPLRELLVRNPRLDAECIDDVILGCANQAGEDNRNVARMATLLAGLPQSVSGTTINRLCGSGLDALGFAARAIKAGDGDLLIAGGVESMSRAPFVMGKAASAFSRQAEMFDTTIGWRFVNPLMAQQFGTDSMPETAENVAELLKISREDQDSFALRSQQRTAKAQSSGILAEEIVPVVLKNKKGVVTEIQHDEHLRPETTLEQLRGLKAPFRANGVITAGNASGVNDGAAALIIASEQMAAAQGLTPRARIVAMATAGVEPRLMGLGPVPATRRVLERAGLSIHDMDVIELNEAFAAQALGVLRELGLPDDAPHVNPNGGAIALGHPLGMSGARLALAASHELHRRNGRYALCTMCIGVGQGIAMILERV

SEQ ID NO: 11 - protein, 400 aa, Pseudomonas putida
MHDVFICDAIRTPIGRFGGALASVRADDLAAVPLKALIERNPGVQWDQVDEVFFGCANQAGEDNRNVARMALLLAGLPESIPGVTLNRLCASGMDAVGTAFRAIASGEMELVIAGGVESMSRAPFVMGKAESAYSRNMKLEDTTIGWRFINPLMKSQYGVDSMPETADNVADDYQVSRADQDAFALRSQQKAAAAQAAGFFAEEIVPVRIAHKKGEIIVERDEHLRPETTLEALTKLKPVNGPDKTVTAGNASGVNDGAAAMILASAAAVKKHGLTPRARVLGMASGGVAPRVMGIGPVPAVRKLTERLGIAVSDFDVIELNEAFASQGLAVLRELGVADDAPQVNPNGGAIALGHPLGMSGARLVLTALHQLEKSGGRKGLATMCVGVGQGLALAIERV

SEQ ID NO: 12 - protein, 394 aa, Ralstonia eutropha
MTREVVVVSGVRTAIGTFGGSLKDVAPAELGALVVREALARAQVSGDDVGHVVFGNVIQTEPRDMYLGRVAAVNGGVTINAPALTVNRLCGSGLQAIVSAAQTILLGDTDVAIGGGAESMSRAPYLAPAARWGARMGDAGLVDMMLGALHDPFHRIHMGVTAENVAKEYDISRAQQDEAALESHRRASAAIKAGYFKDQIVPVVSKGRKGDVTFDTDEHVRHDATIDDMTKLRPVFVKENGTVTAGNASGLNDAAAAVVMMERAEAERRGLKPLARLVSYGHAGVDPKAMGIGPVPATKIALERAGLQVSDLDVIEANEAFAAQACAVTKALGLDPAKVNPNGSGISLGHPIGATGALITVKALHELNRVQGRYALVTMCIGGGQGIAAIFERI

SEQ ID NO: 13 - protein, 406 aa, Rhodococcus sp.
MAEVFLVDGARTPQGRYGGALAGVRPDDLAGLVVAEAARRAGIPGDAVDEVILGAANQAGEDNRDVARMAVLLAGLPDSVPGYTVNRLCASGLTAVASAAHTIRSGEADIVIAGGVESMTRAPWVMAKPGTPWARPGEVADTSLGWRFTNPRFTAADRDVPAGAGPDVRKVTLSMGETAEEVAALEGVTRAESDAFALRSQERAIAAVDAGRFEREIVPVPVRDGELAADETPRRGTTLEKLGSLKPVFRTGGIVTAGSSSSLSDGAAALVVASEAAVEKYGLTVRGRIVTSASAGIAPNVMGLGPVPATRKALARANWSISDLGAAELNEAFAAQSLGVIRQLKLDESIVNADGGAIALGHPLGCSGARILLTLLGRMEREGARRGLATLCVGVGQGVAMLIEAP

SEQ ID NO: 14 - protein, 327 aa, Penicillium chrysogenum
MSAPGAGHEFPAQEVSWQKRDVLLFANSIGVKADELHFLYELHPNFAVFPTYSLILRMSKNTSDFRTIALTPKPLAFKLTDQEVTDFYARQKAVHIPGVPDLDHRHGVDGQRKITILKPLPTTSAGRKFELRNKVIGVYDKGKPGTVIETEQSIVDKESGEVYSKVVSSGFLVGQGGWGGPKGPSTVNYAPPEGRAPDATHVVQSNSETAHLYRLNGDYNPLHATPEPGQKMGFGGIIIHGLFSWNSAAHGILREFGGSNPANMKEFQARFASPVRPGDKLTTEIWRMGNIQDGYEEIRFVTKNDKGRVVLSNGRCLLKVTGVKSKL

SEQ ID NO: 15 - protein, 901 aa, Penicillium chrysogenum
MSELRFDNQTVVVTGAGGGLGKAYALFFASRGANVVVNDLGASHKGEGKSGKAADVVVEEIRAAGGKAVANYDSVENGDAIIETAIKAFGRIDILLNNAGILRDISFKNMKDADWDLINRVHTYGAYKCARAAWPHFRKQKFGRVINTASAAGLFGSFGQANYSAAKLGQVGFTETLAKEGAKYNIIANVIAPIAASRMTATVMPPDVLENLKPDWVVPLVAALVHSSNTTETGGIYEVGGGHVAKLRWERAKGALLKTDDSLTPGAIARKWNDVNDFSQPEYPTGPADFMAFLEDGLKTPSAQPGQEPDFKGRVALVTGGGAGLGRAYCLQFAKLGASVVVNDLVDPEPVVQEIKKLGGKAVGNKASCEDGDAVVKSAIDAFGRIDILVNNAGILRDKAFTNMDDNLWNSVVNVHLRGTYKVTKAAWPYFLKQKYGRVVNTASTSGIYGNFGQANYAAAKLGILGLSRTLALEGAKYNIKVNTIAPNAGTNMTRTIMPEEMVQAFKPDYVAPLVVLLCSDMAPEPSTKGLFECGSGWFGRTRWQRTGGHGFPVDVKLTPEEVVRNWKQIINFDDGRADHPEDGQAGAEKIMANMSNRVHGDTSTENETLKNIKKAKALSSEGTPFNYEDRDVILYNLSLGAKRTDLPLVYENNDQFQALPSYGVVPWFNTATPWNMDDLVKDFSPMMLLHGEQYMEVRKFPIPTTANTLTYPKLIDVIDKGNAAIVVAGYTTKDAKTGEDLFYNESSVFIRGSGGFGGSPKPTAVRPKAATAAYKAPQRQPDAVVEEKTSEDQAALYRLNGDRNPLHIDPEFSKVGGFKTPILHGLCSLGVSAKAVFSKYGPYKNLKVRFAGVVLPGQTLKTEMWKEGNTVLFQATVVETGKPAITGAGAELLEGAKAKL

SEQ ID NO: 16 - protein, 319 aa, Penicillium chrysogenum
MLNSTLRFVSLRRGPTVARNFCSTSAVRAAEVKSLGVVGAGQMGLGIALVAAQKANVPVTLVDTSQASLDKGLKFADKLLEKDVAKQRLTREAADEARGLISTSLTLDGLSAVDFVIEAVPEIPDLKTKIFASLAQIAPKHAILATNTSSISITKIAAATSADPTDLQASSRVISTHFMNPVPIQKGVEIIRGLQTSEETMDTAIAFVQRMGKVASVSADTPGFLANRILMPYINEAVICLETGVGQREDIDNIMKTGTNVPMGPLVLADFIGLDTCLAIMNVLHQDTGDSKYRPAGLLRRMVDAGWLGKKSGKGFYDY

SEQ ID NO: 17 - protein, 335 aa, Penicillium chrysogenum
MATEYPHRIALLGLGTIGLSMLAMHLRRPDTSITVYDPRPNYESQIRSTLPSLLDCPESTTLIDDLLRTSRLKLASTVAEAIQNANIIQEQSPEVTASKQALWKEVAGLTGPDVHLWSSSSGISASVQASGCEAADRVAERLLVAHPFNPPHLMPLIEIVPGPETNPERVEFVRKYFGDVPGPRASGGDQSASQHYRPITLHKEIPGFVGNRLAFALLREACYLVGEGVVSAKDLDSLVTASLGPRWAGSGVFESYHAGGGEGGIGAFLQKLTPTIQDVWGELGQIDIQGEQTWKDVVVKQTEDAYGPYTPETRKKKEEMLRDVVELQKKKWGEL

SEQ ID NO: 18 - protein, 505 aa, Acinetobacter sp.
MTHPIKKIAIIGVGVMGSGIAQIAAQSGHITYLYDAKAGAAQQAKQQLAITFQKLLDKNKITTEYADAANANLLIANELHDLKDCDLIVEAIVERLDIKQSLMSQLEAIVPETTILASNTSSLSITAIASNCKHPERVAGYHFFNPVPLMKVVEVIQGLKTDPKHIETLNQLSRVLGHRPVVAKDTPGFIINHAGRAYGTEALKILNENVTDISEIDRILRDGVGFRMGPFELMDLTGLDVSHPVMESIYHQYYEEARYRPNSLTKQMLEAKQLGRKVGQGFYDYRTGSKTGETSAKVAERLTLYPKVWIAADFEDDKQLLINYLTTHNIQLDVGAKPQADSLCLLACYGEDTTHAALRLNVNPAHSVAIDMLYGIEKHRTLMPSLITEVTYSHAAHSIFNLDGAMVSTIGESIGFVAQRILAMVINLGCDIAQQAIASVDDINAAVRLGLGYPFGPIEWGDEIGSNKILLILNRITALTSDPRYRPSPWLQRRVALNLPLTFTT

SEQ ID NO: 19 - protein, 282 aa, Clostridium kluyveri
MSIKSVAVLGSGTMSRGIVQAFAEAGIDVIIRGRTEGSIGKGLAAVKKAYDKKVSKGKISQEDADKIVGRVSTTTELEKLADCDLIIEAASEDMNIKKDYFGKLEEICKPETIFATNTSSLSITEVATATKRPDKFIGMHFFNPANVMKLVEIIRGMNTSQETFDIIKEASIKIGKTPVEVAEAPGFVVNKILVPMINEAVGILAEGIASAEDIDTAMKLGANHPMGPLALGDLIGLDVVLAVMDVLYSETGDSKYRAHTLLRKYVRAGWLGRKSGKGFFAY

SEQ ID NO: 20 - protein, 319 aa, Clostridium kluyveri
MDIKNVAVLGTGTMGNGIVQLCAESGLNVNMFGRTDASLERGFTSIKTSLKNLEEKGKIKTNISKEILKRIKGVKTIEEAVEGVDFVIECIAEDLELKQEVFSKLDEICAPEVILASNTSGLSPTDIAINTKHPERVVIAHFWNPPQFIPLVEVVPGKHTDSKTVDITMDWIEHIGKKGVKMRKECLGFIGNRLQLALLREALYIVEQGFATAEEVDKAIEYGHGRRLPVTGPICSADLGGLDIFNNISSYLFKDLCNDTEPSKLLKSKVDGGNLGSKTGKGFYNWTPEFLQKKQNERIQLLMDFLEKDKNDKSIERNI

SEQ ID NO: 21 - protein, 475 aa, Escherichia coli
MMINVQTVAVIGSGTMGAGIAEVAASHGHQVLLYDISAEALTRAIDGIHARLNSRVTRGKLTAETCERTLKRLIPVTDIHALAAADLVIEAASERLEVKKALFAQLAEVCPPQTLLTTNTSSISITAIAAEIKNPERVAGLHFFNPAPVMKLVEVVSGLATAAEVVEQLCELTLSWGKQPVRCHSTPGFIVNRVARPYYSEAWRALEEQVAAPEVIDAALRDGAGFPMGPLELTDLIGQDVNFAVTCSVFNAFWQERRFLPSLVQQELVIGGRLGKKSGLGVYDWRAEREAVVGLEAVSDSFSPMKVEKKSDGVTEIDDVLLIETQGETAQALAIRLARPVVVIDKMAGKVVTIAAAAVNPDSATRKAIYYLQQQGKTVLQIADYPGMLIWRTVAMIINEALDALQKGVASEQDIDTAMRLGVNYPYGPLAWGAQLGWQRILRLLENLQHHYGEERYRPCSLLRQRALLESGYES

SEQ ID NO: 22 - protein, 320 aa, Euglena gracilis
MMSRNVFTCCRAIRTYATAPGLSTVGVVGMGAMGHGIAQMTAAAGYKVVAVDIDANMLSKGIKAVEDSLSKVAAKAVKDGKADKATAEKNAADVRSRITTSGDIGALSSCDLVIESIIEDLNIKKKFFADLGKVAGANAILASNTSSFPITQLGEASGRTSNFLGLHFFNPVQMMKLVEVIKTKDTKEDVYKLGFAFSKSIGKEPVACGDTPGFIVNRLLVPFLAQGLLMLDRGVASVQDIDVAMMYGAGMPMGPLTLADYVGLDVCMHILEGWTSQYPNEPAFVIPQPLKAKVAAGKLGRKTGEGFWKWEGDKPVAPAA

SEQ ID NO: 23 - protein, 505 aa, Pseudomonas putida
MAALASNVQVAVIGAGAMGAGIAQVAAQAGHPVKLYDNRPGAAAQAVTGIDRQLARLVDKGKLLAAERETINARLCPVDTLEALADAGLVIEAIVENLQVKQALFSQLETLCAADCILASNTSSLSITSLAAGLERPQHVVGMHFFNPAPLMALVEVVSGLATDPAVAACIYATAQAWGKQPVHARSTPGFIVNRVARPFYAESLRLLQEGAADCASLDALMRDSGGFRMGAFELTDLIGHDVNYAVTCSVFDAFYGDFRFQPSLVQKELVDAGHLGRKTGQGFYRYAEGVERPQPAELHSSACAEACVVEGNLGVMQPLVERLRQSGIAVTQRAGSGLIQVGDATLALSDGRLASQRAREDGLRNLVLLDLALDYSSATRIAISWSADTSDSARDQAVALLQRAGLKVTGVADLPGLVVLRTVAMLANEAADAVLQGVGSAADIDLAMRAGVNYPCGPLAWAANIGIAHTLRVLDNLQCSYGESRYRPSLLLRRCEAKGGTLHD

SEQ ID NO: 24 - protein, 246 aa, Ralstonia eutropha
MTQRIAYVTGGMGGIGTAICQRLAKDGFRVVAGCGPNSPRREKWLEQQKALGFDFIASEGNVADWDSTKTAFDKVKSEVGEVDVLINNAGITRDVVFRKMTRADWDAVIDTNLTSLFNVTKQVIDGMADRGWGRIVNISSVNGQKGQFGQTNYSTAKAGLHGFTMALAQEVATKGVTVNTVSPGYIATDMVKAIRQDVLDKIVATIPVKRLGLPEEIASICAWLSSEESGFSTGADFSLNGGLHMG

SEQ ID NO: 25 - protein, 284 aa, Rhodococcus sp.
MTSTAPKNVGVVGGGRMGAGIAQVFATLGSTVIIAESGDREAAVKRVSDGLDRAHERGKLGDVDPATILGRVSTVAAPDALPPALDLVVEAVPELVDLKLSVLSLVEKTVSPTTVIASNTSSISIAELGSALGDPARLIGMHFFNPVPASSLVEIVRAPATDAGVVEKVREWVAQLGKTEVLVNDSPGFATSRLGVCLGLEAIRMLEEGVADAESIDRAMELGYRHPMGPLRSTDLVGLDVRLAIAEHLAKTLGDRFAPPALLREKVAKGELGRKTGQGFFTWS

SEQ ID NO: 26 - protein, 699 aa, Rhodopseudomonas palustris
MSEVVTRATQDQVAIVTVDSPPVNALSAAVRRGILENVNAAVADPAVQAIVLVCAGRTFIAGADITEFGKPPQPPALNDVIAALENSPKPTIAAIHGTALGGGLEVALGCHFRVAVKEAKLGLPEVKLGLLPGAGGTQRLPRAVGPELAVQMIVGGSPIGAAEALKHGLVEEVVENLVAGAVAFAKKVLAEKRPLRRLRDDDSKLAAAKADRSIFTNAVAAMTKKARGLEAPFACADAIGAAIDLPFEEGLKKEREGFMKLVVSDQSKAQRYAFFAEREAAKVDGVPDGTKPRPVSRVAIIGAGTMGGGIAMSFANAGIPVTLIETGEEQLKRGLGIMQKNWEATAARGGLPPDAPAKRMALITGLVGLENVKDADLIIEAVFETMAVKKEVFTAVDAHAKPGAVLASNTSYLSIDEIAATTKRPQDVLGMHFFSPANVMKLCEIVRGAKTAPDALLTAVSIAKKIAKVPVVVGVCDGFVGNRMLAARSKQSEKLLFEGALPQQVDAVVTKFGMPMGPFAMGDLAGLDIGWRSRKDRGIKSEIADALCEAGRFGQKTGKGYYKYEQGSRAPMPDPEVETLINDTLAKLGLKRRDITDEEILERMVYPMINEGARILEEKIAARPSDIDVVWLYGYGWPIYRGGPMHYADSVGLKHIAERLSAYAKATNDPSLEPAPLLARLAAEGKTFASLTQPSKAAA

SEQ ID NO: 27 - protein, 278 aa, Penicillium chrysogenum
MSLLTTYTTQNTTKIAHLTISHAQKLNSLTTPLLTSLTQTLSKLSNTNLHAITLTGAGQKSFIGGADLNELSTLRNAPTARKFITSVHETCTAIRTCPVPVIARINGFALGAGLEIAAACDLRVAAKGAVFGMPEVRLGIPSVVEAALLPGLIGWGRTRQLLLLGGMISASEALRWGLVERVVEDEELDLAVAEWTSEIGRNGPLAVRRQKALISRWEELSLAGGIEAGIEAFGECFDGDCGTEPGRMIGEFFREKERSKARIEARNKVVAGSKGEEG

SEQ ID NO: 28 - protein, 244 aa, Penicillium chrysogenum
MTEIPTFHNLSLERHGNVFVLTMQKPPENRLNSSYCQEMIRAYRSVERILGSDSEGAVITRGNDAKFWCTGLELDESDSNPFANTDGFYPLIHTILDFPFPTVALLTGHTFGGACPLALAHDYRIMNSRRGFISMPPVNLGLHFDGIGSLPRLKLRPQVARKMLLEAHRWTGPEALEDGIVDAVAEPEDMLNVALELGAKWAPKAKMGVYALLRQELWGDAIKKFQRISYVHSRVTSAPAKVKI

SEQ ID NO: 29 - protein, 300 aa, Penicillium chrysogenum
MAPSDRLTQVNEHLNYPAGLLAGQVAIITGAGQGIGAEAARLFANEGAKVVVADIDSKKANAVADAINSAKAGRALAVVGDVLDSNYITELVKKTAEFGNGKIHIIVNNAGFTWDGVIHKMTDKQWETMLAVHNTAPFQLVRAAAPYFRVKDQEPRVVINISSTSGVHGNAGQANYAVAKAGVVGLTRTIAKEWGPSFGVRSNTIAFGFVTTRLTAAKEEGAFITTPDGTKVALGIPGKQLATKKGSADQEKKAAPTYPDIPLGRPATPEEAARAVLGVASPWFSYVNGETIRVTGGRNM

SEQ ID NO: 30 - protein, 327 aa, Penicillium chrysogenum; identical to SEQ ID NO: 14

SEQ ID NO: 31 - protein, 901 aa, Penicillium chrysogenum; identical to SEQ ID NO: 15

SEQ ID NO: 32 - protein, 293 aa, Penicillium chrysogenum
MFARQCTRLATSRTSAPLTSYLARVRGYSSAAGSYEHILTSTPKPGVGLITLNRPKALNALCSPLFKELNEALSNYDNDKSIGAIIITGSEKAFAAGADIKEMAPLSFSAAYSDNFIAPWSHLATSIRTPVIAAVSGYALGGGCELALMCDILYCSENATFGQPEIKLGTIPGAGGSQRLTRAIGKSKAMELILTGKNFSGKEAGEWGVAAKVVPGGKEELLEQAYKTAETIASYSRVAVVAGKEVVNKSQELSLKEGVEYERRLFHALFGSKDQKIGMTAFAEKKKPEWSHE

SEQ ID NO: 33 - protein, 261 aa, Acinetobacter sp.
MIPDQDNFVEIDFSIEQIAIVKINRPASKNALNTEVRKQLAQAFTELSFNDQINAIVLTGGEDVFAAGADLKEMATASSTDMLLRHTERYWNAIAQCPKPVIAAVNGYALGGGCELAMHTDIIIAGKSATFGQPEIKVGLMPGAGGTQRLFRAVGKFHAMRMIMTGVMVPAEEAYLIGLVSQVTEDSQTIPTAIKMAQSLAKMPPIALQQIKEVALMSEDVPLNAGLTLERKSFQLLFSTEDKNEGINAFIEKRKPSYHGK

SEQ ID NO: 34 - protein, 136 aa, Aeromonas salmonicida
MNTLPLEIGQKASLTKRFGAAEVEAFAGLSEDFNPLHLDSAFAATTPFERPIVHGMLLASLFSGLLGQQLPGKGTVYLGQSLSFKQPVFVGDEVTAEVEIIAMRSDKPIITLATRILAAGGALALAVTGEAVVKVG

SEQ ID NO: 35 - protein, 259 aa, Clostridium kluyveri
MEFKNIILEKDGNVASITLNRPKALNALNAATLKEIDAAINDIAEDDNVYAVIITGSGKAFVAGADIAEMKDLTAVEGRKFSVLGNKIFRKLENLEKPVIAAINGFALGGGCELSLSCDIRIASSKAKFGQPEVGLGITPGFGGTQRLARAIGVGMAKELIYTGKVINAEEALRIGLVNKVVEPDKLLEEAKALVDAIIVNAPIAVRMCKAAINQGLQCDIDTGVAYEAEVFGECFATEDRVEGMTAFVEKRDKAFKNK

SEQ ID NO: 36 - protein, 257 aa, Clostridium kluyveri
MTYKTLLLEKQNGITIIKMNTPHNLNAISQQSVEDLFAVLQVIKNDDNCRVVILTGEGKGFIGGADIKHMACLDAIEGGQFCFAVSKCTLEMEKMGKVFIAAVNGFALGAGLEVALGCDIRIFSKHAKIGFPETGLGVIPGAGGAQRLQRLVGIGKASEIIFTGDIIGADDALRFGIANQVTEPESLMDTAMSMAEKILTKSPVGTRLAKEALQKGRDTDLEKALEYDKNLFGLCFSTEDKKEGMAAFIEKRKPVFK

SEQ ID NO: 37 - protein, 255 aa, Escherichia coli
MSELIVSRQQRVLLLTLNRPAARNALNNALLMQLVNELEAAATDTSISVCVITGNARFFAAGADLNEMAEKDLAATLNDTRPQLWARLQAFNKPLIAAVNGYALGAGCELALLCDVVVAGENARFGLPEITLGIMPGAGGTQRLIRSVGKSLASKMVLSGESITAQQAQQAGLVSDVFPSDLTLEYALQLASKMARHSPLALQAAKQALRQSQEVALQAGLAQERQLFTLLAATEDRHEGISAFLQKRTPDFKGR

SEQ ID NO: 38 - protein, 257 aa, Pseudomonas putida
MPRYLDVQAPENGVQLITLQRPEALNALCTELLAELATALDAAARDDQIGVVVLTGSRKAFAAGADIREMAERDLVGILNDPRVAHWQRIAAFAKPLIAAVNGYALGGGCELVMCADIVIAGSDARFGQPEINLGIIPGAGGTQRLLRAVGKPLAMQMVLTGEAITARHAQQAGLVSEITQPEFTVERAMQIARNIAAKAPLAVRLAKEALLKAGDTDLASGLRFERHAFTLLAGTADRDEGIQAFQEKRPARFQGR

SEQ ID NO: 39 - protein, 263 aa, Pseudomonas putida
MTFQHILFSIEDGVAFLSLNRPEQLNSFNAAMHLEVREALKQVRQSSDARVLLLTAEGRGFCAGQDLSDRNVAPDAEVPDLGESIDKFYNPLVRTLRDLPLPVICAVNGVAAGAGANIPLACDLVLAGRSASFIQAFCKIGLVPDSGGTWLLPRLVGMARAKALAMLGERLGAEQAQQWGLIHRVVDDAALRDEALTLARQLASQPTYGLALIKRSLNASFDNGFDEQLELERDLQRLAGRSEDYREGVSAFMNKRTPAFKGR

SEQ ID NO: 40 - protein, 699 aa, Rhodopseudomonas palustris; identical to SEQ ID NO: 26

SEQ ID NO: 41 - protein, 242 aa, Rhodococcus sp.
MNTLKIEDRDDRMVVTLHRPAQRNAINAEMIGELHQVCASLEATPKPMLLTGEGDHFAGGADIAELRERGRDEAFAGINRNLFDRIAKLPMPTVAAVSGYALGGGAELSYACDIRIATETAVFGNPEPGLGIMAAAGASYRLPELVGTSVAKQVLLGGRNLDAQDALRSGLVMSVVAPGEHIDAAHKVIDRITRSAPLALKLTKMIVDAPGSHPFADDIAQAVLFESRDKHDRMTAFLEKKK

SEQ ID NO: 42 - protein, 689 aa, Penicillium chrysogenum
MPDFTDNLRPSQPDGPTTLARERQKSNIATEELGQHLLGSDGFLVRQARILPIIQQEPLFSKDQQQNLSRPERFKLGVARAKLLRQMKDTHKWSHLEYQMAEYLVDDVSPYFLHMEMFITTIREQASEEQQAHWLPLIELWKIIGAYAQTELGHGSNVRGLELEARWDNRTKEFVLHSPTLTASKWWNGSLGRLANHAIVVAQLLLPDPSSPDQYVSHGPHPFIVQVRDMKTHQPLNGIVVGDIGPKYGYITMDNAYMLFDQFRIPHSAMLSRYSKVDLNTGIYTKPEKPALVYGSLTYVRSNMVHRARLVLARAVTVAVRYSSVRRQFQDRDGDKTGPEMSVLDYPTVQIRILPLLATTFALHYTGLAMQTVYKNARQDIEEGNFNSLAHMHSMSSGLKSLCTIFAADGIETCRRAMGGHGFGGGSGLIQVNNDYLSKPTVEGDNWMITQQVAAYVIKKMTAAVGSPDTPGIDETDARFKEFIRNKRRPESEKRTYDILNSDLDIVKSFELRATAMASSTKLIRVIKKRNWNSLLIQLHKLSRAQSESIIVATFFDALSNDKTLSAPTKNVLWDCYRLFALYSMENESFEFLRTNAVSQTDLDSLASRVQDLMARIRPHAVTLVDSWMIPDYLLDSALGRYDGRVYEDLFNRAHRLNPLNRITFNPNYWEDEIVKGSGDNGRGILSKL

SEQ ID NO: 43 - protein, 425 aa, Penicillium chrysogenum
MSVSNVPFADPLWLNRKHSPYYKDSHRKLQKEVRQYVDEHISPFCEEWEKQGFVPPEAQKRHAELGYTAVASFPLAADYLDGQRLPGDINPYEWDGFHDIVVIDELARCGYLGIVWALGCGNSIGGPPIINFGNEEQKRRFLPDMLKGKIRFCLGVTEPDAGSDVAGITTVAERKGDAYIVNGAKKWITNGIFADFCTAAVRTGGSGTHGISALVIPMKAPGVICRKIENSGVHASGSTYIEFDQVEVPVDNLLGEENKGFPVIMNNFNHERLWLACTSLRMARVCAEDAYQHAITRETFGKRLIENQIIRSKFSAMARSLDSNYAWMEQLVYIAEIAKKEGTDAGTGGLFANLKVLAGQTLEKVNRESQQVMGGLGYSKNGRGSRIEQVSRDVRVMVVGGGSEEILSELAVNQEIKAMKKQSKL

SEQ ID NO: 44 - protein, 605 aa, Penicillium chrysogenum
MAAQSRVPATAESGTFTQLGPLPNTYTSDISLQRMLGWYLPAQTLKLIEPHLAQLGEEAVSPQVFAWNADAETNLPYVKKYNVWGQRYAYDRLVTTDGWKQLGKWGAKHGVVSLGYDHTYGVYRRTAQYAAVYLYAPSSAMYRCPMSMSDGAALTSGQWMTERAGGSDVQNTETWATYAPLPQESKTSDVLAEGDYLISGFKFFSSATDANVAFLLAKTDSGKLSTFIAPLRKTSIGADGKPEETSNGVRIHRFKNKLGTKELPTAELELKGMRAHLVGELDQGIVTIAPLLNTTRIQTLLGTLSTWRRAISITKNFAKSRTTVGEPLWLIPMHLRLLADVEVKHRGAINLAFFTIAVMGLIENPSSPARHAHMPRDPTEAKVVFRVLTATSKGVVSKMSMVGVQECQEAIGGVGYIDEPDEPEFNISRLLRSAAVYPIWEGTTNVLASELVRFLMKGDNLSILSGWLGHVVSLIRTPSLAGALKQAMASYLSRVTSTRPQAALLADARRVMFTFAWILSGALLTLDAERDEDEVAMEIARRWVLLGEGGVGEFVYRDIAKPYQCFNLRSGRDEHTRLDCKIAWGVELPGKIVFGHRSLSESSKL

SEQ ID NO: 45 - protein, 425 aa, Penicillium chrysogenum
MMNRSLLRAAARSIQAGPTSVAGRRYASSAVFNWEDPLAAAELFTDEELAIQDTARQYCQDKLAPRVLEAYRNEDYDRRILEEMGDLGLLGASIEGYGCAGVSTVASGLITKEVERVDSGYRSGMSVQSSLAMTGIYEFGTEEQKQRFLPSLAKGTLAGCFGLTEPNHGSDPGSMETVAREHPTQKGMYLLSGSKTWITNSPIADVALVWAKLESTGKIRGFIVERERATPGSYETPAIKNKSALRASITGMIQMDNCPVPAENMLPEVEGLKGPFTCLNSARLGIAFGAMGALEDCLARAREYSLERKQFKGNPLAKYQLIQMKLANAATDAAYGTLAAVQVARLKDAGKATPEMISMIKRQNCDRALANSRILQEVFGGNAASDEYHIARHVANLFVVQTYEGQSDIHALILGRAITGKQAFV

SEQ ID NO: 46 - protein, 633 aa, Penicillium chrysogenum
MSSSQPATADSGYITDPGPLENTYTSDPSLQRALAWYLPSATLQSVQPHLTQFGAEAISEQVREWSADAERNVPYVKSHNVWGKRYDYDRLVTTEGWKQLGKWGARNRIVSAGYDKSLGVDRRTVQYALNYLYSPSSGLYSCPISMTDGAAFILSSRINKLPSTHPFHTAFQGLISEKDDHWTSGQWMTERAGGSDVQNTETWATYSPLASSSGSEPLGDGDYLISGFKFFSSATDANLALLLAKTPSGKLSTFLAPLRRTVVGGDGVSRVVSNGVRIHRLKNKLGTKELPTAELELKDMRAHLIGEIDQGIVTIAPLLNVTRLHTFVGSLAGWRRAISITKSFAKARTTVGEPLWLIPMHLRLLADMEVKHRGAMNLAWFTVALFGVVEDRTPSSNKIAHLPQPGKEAEVVFRTLTATAKAVISKMATAGIQECQESMGGVGYMDEADEPEFNISRILRNNAVNSIWEGTTNVLASEFVRFLIKKDNLKIFGTWLDRTLALIQSVDLRNALTAAWLALHARFMTQDPATTVADGRRFMFTVAWILSGALLALDTERDNDPVTAEIARRWILSAEGGVGEQVFHDIVTVSGTASATSGGEEHLQWDCRIAWGVDLPANRASGHRSLQKAGSKL

SEQ ID NO: 47 - protein, 695 aa, Penicillium chrysogenum
MPSPPPDWVKALKPSGPQGSELLHQERAQSNVDVERLSELLHTKETLERRASLLALLQPEKVFDKSQNHSLGRVERLQRSLAKAKRLQQLAEEHKWSMQELHAANDLIGEPTPYGLHASMFLVTLREQGTPEQHKLFLERAEKYEIIGCYAQTELGHGSNVRGLETTATWNSNDKTFTINSPTLTASKWWIGSLGRTANHAVVMAQLFIDGKNYGPHPFVVQVRDLETHQPLDNVYVGDIGPKFGYNTMDNGFLLFNNVKIPHVNMLARFCQVDKETNQYAKPAMPSLVFGTMTWVRANIVLDAGGVLARGVTIATRYCAVRRQFQDRDADPHAGETQVLNYKMVQVRLLPLLASMYALHFTGRGMMRLYEENQSRMKAASSPDQESRGAGPEQLRAGANLLADLHATSCGLKALASTTAGEGLEICRRACGGHGYSSYSGIGPAYADYLPTLTWEGDNYMLTQQVARYLLKSARAVLAGKPARNDTSQILQAYLDRRDKGASFDVLDEDKDIVAAFGWRTAHLTFEALKHRDAEQRSWNSLLVDFWRLSTAHSQYLMVKNFYEAVSSPELSGALDPETKGLMHQLFRLFSLHTLEREAAEFFSSGAVTVRQITLTRTTAVLKLLDDIRPHAVRLVDAWAIPDWQLDSSLGRYDGKVYEDLFRRASEENPVNELVFDPYPWNSALLKNEPAKSKL

SEQ ID NO: 48 - protein, 542 aa, Penicillium chrysogenum
MAKTFSKEDVASHSKGDSPWIIIDEDVYDVSKFQEEHPVLQRVAGKDASKQFWKYHNEGILKKYKGQLQIGSLDTKKAAPAPPTPAPAPKKAAPEPKSTASSSSVTPPATGAPQDPYGELIPFADPSWYQGYASPYFNESHAALRDEVRQWVESEIEPYVTEWDEAKEVPAHIYKQMGERGYLAGLLGVHFPEKHTPHRVKSVSPDRWDLFHEMLLTDELSRAGSGGLVWSLIGGYGIGCPPLVKFGKKPLVDRILPGILAGDKRICLAITEPDAGSDVANLGCEAKLTEDGKHYIVNGEKKWITNGIYSDYFTTAVRTGKDGMNGLSVLLIEREAGGVSTRRMDCQGVWSSGTTYVTFEDVKVPVENLIGKENQGFKVIMTNFNHERIGIVIQCVRFSRVCYEESMKYAHKRKTFGKRLIDHPVIRMKLAHMARQIEATYNWLENIIFQCQSMEDTEAMLKLGGAIAGLKAQSTQCFEFCAREASQIFGGLSYSRGGQGGKIERLYRDVRAYAIPGGSEEIMLDLSMRQSLRVHGMFGMKL

SEQ ID NO: 49 - protein, 438 aa, Penicillium chrysogenum
MADTLRPATAPYSEPLLPQLDVRNPYYTDLHHNLRATVREYVDTYISPYAAEWEEAGQVPEAVRRRHCKLGYSIVHPLTSEEDSAGISLPGNVPREKWDTWCSLIVSDELTRVGYVGVIWGLGGGNGIGCPPVARFGNAEQRKKWLPGVARGDIRFCLGITEPDAGSDVANIQTTAQRDGNHYVVNGSKKWITNGIWADYCTAAVRTGGPGRSGISLLVIPLATAGVTRRRMHNSGVNASGSTFIEFEDVRVPVENLVGQENKGFPLIMSNFNPERLALACASLRLARVCAEDAYNYAIKRETFGSALIEKQAIQSKIFKFGLMIEPAYAFMEQLVNILELTKDRPSDDVNIGGMTALLKVMSTRALEKSVREAQQIMGGAGYNKAGKGARIEQISRDARVHVVGGGSEEIMAGLALREETKAIRTRRKALEKRQSKV

SEQ ID NO: 50 - protein, 453 aa, Penicillium chrysogenum
MNFDLPADLKTHLESIDSFIHSTILPLQHSNDNNRFFDHRREYERTDWENNGNPRKEWEELLGEARTLADSSGLYRFALPRVYGGQSHPDVNLWMSAIRYHLSSNAVYGGGLGLANDLQNEHCIVGNFPDVLMLHHFGNEQQRNTLIPARLRGEFRTTFGLTEPDHGSDATFMSTTARPTRGGFEIKGAKKWQTGAHHCTHFLIFARTSGKAGSAQGITAFLVPRDTRGVRIVSYEWTLNMPTDHATVELNSVWVPESAVLGSIDQGLAIAQTFVHENRIRQAASSCGAARYCLDRSIDRARARKIWGEGKSLADNQAIQFPVVELMTQVEMLRLFILKTSWEMDRIVAECQSSKAQRAPWVEIEGRLSDQVAMCNFWANRLCCQAADRAIQIHGGDGYSRHYPFEHIYRHFRRYRITEGAEEIQMRKIGAYIFGFAGPKKREMKHEHSKARI

SEQ ID NO: 51 - protein, 441 aa, Penicillium chrysogenum
MAYNSPNPIPFSEPPYIRGLPSPYITPAHRRFQQACRKFATENLIQHALEWEREGTVPEHVFHTFCKHNMLLPNMPAPLPVDWLKRLGINDILGVKVEDWDYIYTGIYCDEMARSGLSGPSGSLNAGFAFGIAPIYKFGSTELQERFLPELLTGKKRGCIAITEPEAGSDVANITTTAVKSADGQHYILNGSKKWITNGIWSDYATMAVRTGGPGAAGLSVLVVPLKGHPGVSMRRLKVSGQITGGTTYIELDDVKVPVSNIIGKEGDGMRIIMTNFNHERLVIAVGVTRQARVALSAAFSYCLKREAFGKTLMDQPVVRHRLAKAGAELESMWAWVEQILYQLVHLSKEEGDRQLGGLTALAKAKSAMVLNECAQTAVLLFGGNGFTKTGQGELVEAILRDVPGARIPGGSEDVLLDLSVRQLVKLYQAEEKKLSKNAKI

SEQ ID NO: 52 - protein, 439 aa, Penicillium chrysogenum
MYRSQIQRALRSQWPALRQLQCRTGLSPRARAAFSTSGRRDIMGMTGFTDEQLTVREAISHICSRFPNTYWQERDQQEKDPKEFHAALAKDGWLGIALPESLGGAGLGISEATMMMQTITQSGAGMAGAQAIHANVYATQPLAKFGTKEQLETTIPNIINGTWRTCFGVTEPNTGLETLKLTTLASKTDDGYSVTGQKIWITCAQVASKMILLARTTPLEEVKKSSEGLSLFCIDIDRENPGLDLRKIKKMGGRAVDANEVFFDHYKIPANTLIGEENQGFKIILHGMNAERCLLAGEALGLGYAALEKASQYAKDRVVFGRPIGQNQGVAHPLADAFMKLEAAKLATYHAARLYDTNDGSVPFHEIGVACNSAKYLAAEAAFTACERAVLAHGGMGYAVEYDVERYMRECFVPRIAPVSREMILNYVSEKVLDLPRSY

SEQ ID NO: 53 - protein, 446 aa, Penicillium chrysogenum
MSASSRIPPIAQPFVSEHAKRTLDLVEEFVEKDCIPADTVFSAQLGEGEKRWTTTPTVLEGLKEKAKKLGLWNMFLPKNHFTQGAGFSNLEYGLMAELLGKSKVASEATNNAAPDTGNMEVFAKYGNDAQKKQWLAPLLEGKIRSAFLMTEPDVASSDATNIELNIRREGNEYVLNGSKWWSSGAGDPRCAIYLVMGKTDPTNPDTYKQQSVILVPAGLPGITVHRMLTVYGYDDAPHGHGHITFKDVRVPASNMVLGEGRGFEIIQGRLGPGRIHHAMRAIGAAERALEWLIARVNDERKMTFGKPLVAHGVILEWIAKSRIEVDAARLIVLNAAIKIDQGDAKSALKEIAQAKVLVPQTALTIIDRAVQAYGAAGVCQDTPLAYLWAGIRTLRIADGPDEVHLQQLGKRENKARKDAVTAKLNWQREEADRLLAASGFKPKSHL

SEQ ID NO: 54 - protein, 513 aa, Penicillium chrysogenum
MPSETLTRAEVAKHNTEDSLWCIIDHQVYDLTDFVDAHPGGGVVLAQVAGKDATSDFYNLHRQEVLEKYRDQLCIGVVEGEKPEVIRPFPGALSPVPYAEPLWLRPQFKSPYYKETHRNLQKAIREFTDKYVTPEAQEKEQDGSYISQELINRMAETNILAMRLGPGKHLHGRTLLGGVVDGKEFDYLHDMIIVQEMVRANARGFQDGNMAGMAISLTAVQQWLHDPVLKERLNDEVLSGRKKMCLAITEAFAGSDVAGLKTTAEKTPDGKHYIVNGTKKWITNGMFADYFVTGCRTEKGFSVLLIPRGEGVETKQIKTSYSTAAATAFVEFDNVKVPVQNLLGEEHKGFIVIMSNFNHERFMMVAAVVRMSMMVVEETMKWSNQRIVFGKKLIEQPVIRQKIARMISLAESNQAWLESIAYQMCNMTYAQQAKLLGGPIGLLKSHCTQAAGEIASLATNIFGGRGLTQSGMGKVIEMFHRTYKFDAILGGTEEILADLGVRQAMKNFPKSML

SEQ ID NO: 55 - protein, 436 aa, Penicillium chrysogenum
MASIIRALRPLSRNPSVRLAGKRLAAGRPVQSAYAFSTTPRRREVDLSELTPTPITLLSETESLMADSVSKFAVEQIGPKVREMDEAETMDAKVVEQLFEQGLMGIEVPEEFGGAGMNFTAAIVAIEELARVDPSVSVLVDVHNTLVNTAIMKYGDAKAQRTWLPKLTTGTVGSFCLSEPASGSDAFALQTKAEKTADGYKLNGSKMWITNSMEAGVFIVFANIDPSKGYKGITAFIVEKDTPGFSIAKKEKKLGIRASSTCVLNFDDCVIPKSNLLGEEGQGYKYAISVLNEGRIGIAAQMTGLALGAWENAARYVWNDRRQFGELIGNFQGMQHQIAQAYTEIAAARALVYNAARKKEAGQDFVQDAAMAKLYASQVAGRVSSSAVEWMGGMGFVREGIAEKMFRDSKIGAIYEGTSNIQLQTIAKLLQKQYTN

SEQ ID NO: 56 - protein, 429 aa, Penicillium chrysogenum
MASLTLPSLLRTSTRAVRLNRTPALTPCFRSISTKHPKGFIPPSEDDLLELRERVQDFTRREIPADVAARTDEQNEFPAEMWRKMGDAGFLGVTANEEYGGLGMGYQAHCVVMEEISRASGSIGLSYAAHSQLCVNQLSLNGSTEQKERILPGLLSGEKVGALAMSEHSAGSDVVSMKTTAKEVDGGWLLNGTKMWITNGPDADYIVVYAKTEPELGSKGITAFLVEKDFKGFSCARKLDKLGMRGSNTGELIFEDVFVPRENLLGEVNRGVRVLMEGLDLERLVLSAGPLGIMQAALDLVLPYTHVRKQFGAPIAHNQLVQGKLADMYTKLAASRAYTYATARQVDNAAVEPGELTVRTQDCAGAILYAAERATECTLDAIQLMGGSGYINEIPAGRLLRDAKLYEIGAGTSEIRRMVIGRAFNKEYA

SEQ ID NO: 57 - protein, 405 aa, Penicillium Chrysogenum
MFSRSVLQTATRSVRPASARAVPQLGKAPFGRRYVSVYGYTQAKALIYSKYGEPKDVLRLHKHSISAPHATQVNLRLLTAPMNPADVNQIQGVYPSKPPFQTELGNVEPAAVGGNEGAFEVLSTGAGVKNLSKGDWVIMKRTGLGTWRTHAQLDESQLIKVENKEGLTPLQVGTVSVNPVTAYRMLRDFCEWDWMRAGEEWVIQNGANSGVGRAAIQLGREWGIKTLNVIRQRKTPEETEALKQELRDLGATVVITEEEMLNGNFRDMVHEFTRKGREPIRLALNCVGGKNATALAKTLAPDSHMVTYGAMSKQPVALPSGLLIFKNLAFDGFWVSKWGDKNPQLKESTIKDVLQLTRSGKFKDIPVDEVKWNWETEGPELAESVQGTLGGYRSGKGVFTFSGGD

SEQ ID NO: 58 - protein, 373 aa, Bos taurus
MWVCGALCRTRAPAQLGQRLLPESRRRRPASASFSASAEPSRVRALVYGHHGDPAKVVELKNLELAAVGGSHVHVKMLAAPINPSDINMIQGNYGLLPQLPAVGGNEGVGQVVAVGSGVTGVKPGDWVIPANPGLGTWRTEAVFGEEELITVPSDIPLQSAATLGVNPCTAYRMLVDFERLRPRDSIIQNASNSGVGQAVIQIAAARGLRTINVLRDTPDLQKLTDTLKNLGANHVVTEEELRKPEMKSFFKDVPQPRLALNCVGGKSSTELLRHLAPGGTMVTYGGMAKQPVIASVSQLIFKDLKLRGFWLSQWKKDHSPDQFKELILTLCDLIRRGQLTAPACSEVPLQDYLCALEASTQPFVSSKQILTM

SEQ ID NO: 59 - protein, 302 aa, Cavia sp.
MGSWTKCQSCLAPGLLQNRAAIVTGGGTGIGKAIAKELLHLGCNVVIASRKFDRLRAAAEELKATLPPSNKAEVTPIQCNIRKEEEVNNLMKSTLALYGKIDFLVNNGGGQFWSSPEHISSKGWHAVIETNLTGTFYMCKAAYNSWMKEHGGAIVNIIILLNGQPFVAHSGAARGGVYNLTKSLALGWARSGIRINCVAPGTVYSQTAMDNYGDMGKTLFADAFQKIPAKRLGVPEEVSSLVCFLLSPAASFITGQLVNVDGGQSLYCQNHDIPDHDNWPEGVGDLSTVKKMKESFKQKAKL

SEQ ID NO: 60 - protein, 386 aa, Candida tropicalis
MYSVLKQSIRPRLLATHNQFRTMITAQAVLYTQHGEPKDVLFTQSFEIDDDNLAPNEVIVKTLGSPVNPSDINQIQGVYPSKPAKTTGFGTTEPAAPCGNEGLFEVIKVGSNVSSLEAGDWVIPSHVNFGTWRTHALGNDDDFIKLPNPAQSKANGKPNGLTINQGATISVNPLTAYLMLTHYVKLTPGKDWFIQNGGTSAVGKYASQIGKLLNFNSISVIRDRPNLDEVVASLKELGATQVITEDQNNSREFGPTIKEWIKQSGGEAKLALNCVGGKSSTGIARKLNNNGLMLTYGGMSFQPVTIPTSLYIFKNFTSAGFWVTELLKNNKELKTSTLNQIIAWYEEGKLTDAKSIETLYDGTKPLHELYQDGVANSKDGKQLITY

SEQ ID NO: 61 - protein, 379 aa, Clostridium kluyveri
MDFTLTNEQKFVEQMVSEFTENEVKPIAAEIDETERFPLETVEKFAKYGMMGMPFPVEYGGSGTDYLSYIIAVEGLAKSCTSSSTILSAHTSLCAAPIYDWGTEEQKQKYLVPLAKGEKLGAFGLTEPNAGTDAAGQQTTAVLEGDHYVLNGQKIFITNGAYADTFVIFAMTDRSKGTRGITAFIVEKDFPGFSIGKSEDKLGIRASSTTELIFENCIVPKENMLGKEGKGFTVAMHTLDGGRIGIAAQALGLAEGALAEALNYMKERKQFGKALYKFQGLAWMVAELDTKIEAVKQLVYKAAVNKQMGLPYSVEAARAKLAAATVAMETTTKVVQIFGGYGFTKDYPVERMMRDAKITEIYEGTSQVQKMVISANLFK

SEQ ID NO: 62 - protein, 562 aa, Clostridium kluyveri
MNFELTKEQQMIRDNVRKFAEAKIEPIAFQLDEKNIFPEEIVNEMGDLSIMGLPYPKEYGGAGKDVLSYAIAVEELSRVDAGVGVILSAHTSLGTWPIMEFGTKEQKEKYLVPLASGKKIAAFGLTEPNAGSDAGKTETTAVLEGDHYVINGSKVFITNADYADTYVIFAVTTPGLGTKGISAFIIEKGMDGFTFGTHYNKMGIRSSATAELLFKNLKVPKYNLLGKENEGFKIAMQTLEGGRIGIAAQALGIAQGAYEKALSYSKERVQFGKPISRQQSIAFKLADMATKIRAARFMVYSAAVLKQEHKNYGMESAMAKLYASDICLEVVNDAVQIYGGSGFIKGFPVERMYRDAKICTIYEGTNEIQRLIISNDILGKPKKEPIEENKENKVNKAKPITGNRRRVIIKEGSPKEKVDAFLNYIKSENIDINKSEASKGSIADADKVCSIGLGLKDKKDLPLIQSLADTVGAELGCSRPVAEEREWLPLDRYVGISGQKFGGTFYLAIGISGQVQHLKGIENAGIITAINIDEDAPIFKSSDYGIVGDLYEIVPLLIEALK

SEQ ID NO: 63 - protein, 539 aa, Euglena gracilis
MSCPASPSAAVVSAGALCLCVATVLLATGSNPTALSTASTRSPTSLVRGVDRGLMRPTTAAALTTMREVPQMAEGFSGEATSAWAAAGPQWAAPLVAAASSALALWWWAARRSVRRPLAALAELPTAVTHLAPPMAMFTTTAKVIQPKIRGFICTTTHPIGCEKRVQEEIAYARAHPPTSPGPKRVLVIGCSTGYGLSTRITAAFGYQAATLGVFLAGPPTKGRPAAAGWYNTVAFEKAALEAGLYARSLNGDAFDSTTKARTVEAIKRDLGTVDLVVYSIAAPKRTDPATGVLHKACLKPIGATYTNRTVNTDKAEVTDVSIEPASPEEIADTVKVMGGEDWELWIQALSEAGVLAEGAKTVAYSYIGPEMTWPVYWSGTIGEAKKDVEKAAKRITQQYGCPAYPVVAKALVTQASSAIPVVPLYICLLYRVMKEKGTHEGCIEQMVRLLTTKLYPENGAPIVDEAGRVRVDDWEMAEDVQQAVKDLWSQVSTANLKDISDFAGYQTEFLRLFGFGIDGVDYDQPVDVEADLPSAAQQ

SEQ ID NO: 64 - protein, 303 aa, Homo sapiens
MASWAKGRSYLAPGLLQGQVAIVTGGATGIGKAIVKELLELGSNVVIASRKLERLKSAADELQANLPPTKQARVIPIQCNIRNEEEVNNLVKSTLDTFGKINFLVNNGGGQFLSPAEHISSKGWHAVLETNLTGTFYMCKAVYSSWMKEHGGSIVNIIVPTKAGFPLAVHSGAARAGVYNLTKSLALEWACSGIRINCVAPGVIYSQTAVENYGSWGQSFFEGSFQKIPAKRIGVPEEVSSVVCFLLSPAASFITGQSVDVDGGRSLYTHSYEVPDHDNWPKGAGDLSVVKKMKETFKEKAKL

SEQ ID NO: 65 - protein, 303 aa, Mus musculus
MGSWKTGQSYLAAGLLKNQVAVVTGGGTGIGKAVSRELLHLGCNVVIASRKLDRLTAAVDELRASLPPSSSAEVSAIQCNIRKEEEVSNLVKSTLAKYGKINFLVNNGGGQFMAPVEDITAKGWHAVIETNLTGTFYMCKEVYNSWMREHGGSIVNIIVLLNNGFPTAAHTGAAREGVYNLTKSMALAWASSGVRINCVAPGTIYSQTAVDNYGEMGQTLFEMAFDSIPVSALGVPEEISLLARFLLSPAASYITGQLINVDGGQALHTHAFSIPDHDNWPVGAGDLSIVKRIKESFKKKAKL

SEQ ID NO: 66 - protein, 373 aa, Rattus norvegicus
MLVSRRLTGARARAPLLASLLEAWCRQGRTTSSYSAFSEPSHVRALVYGNHGDPAKVIQLKNLELTAVEGSDVHVKMLAAPINPSDINMIQGNYGLLPKLPAVGGNEGVGQVIAVGSSVSGLKPGDWVIPANAGLGTWRTEAVFSEEALIGVPKDIPLQSAATLGVNPCTAYRMLVDFEQLQPGDSVIQNASNSGVGQAVIQIASALGLKTINVIRDRPDIKKLTDRLKDLGADYVLTEEELRMPETKNIFKDLPLPRLALNCVGGKSSTELLRHLAPGGTMVTYGGMAKQPVTASVSMLIFKDLKLRGFWLSQWKKNHSPDEFKELILILCNLIRQGQLTAPAWSGIPLQDYQQALEASMKPFVSLKQILTM

SEQ ID NO: 67 - protein, 380 aa, Saccharomyces cerevisiae
MLPTFKRYMSSSAHQIPKHFKSLIYSTHEVEDCTKVLSVKNYTPKQDLSQSIVLKTLAFPINPSDINQLQGVYPSRPEKTYDYSTDEPAAIAGNEGVFEVVSLPSGSSKGDLKLGDRVIPLQANQGTWSNYRVFSSSSDLIKVNDLDLFSAATVSVNGCTGFQLVSDYIDWNSNGNEWIIQNAGTSSVSKIVTQVAKAKGIKTLSVIRDRDNFDEVAKVLEDKYGATKVISESQNNDKTFAKEVLSKILGENARVRLALNSVGGKSSASIARKLENNALMLTYGGMSKQPVTLPTSLHIFKGLTSKGYWVTEKNKKNPQSKIDTISDFIKMYNYGHIISPRDEIETLTWNTNTTTDEQLLELVKKGITGKGKKKMVVLEW

SEQ ID NO: 68 - protein, 365 aa, Penicillium Chrysogenum
MSKRVTIFDPPEQDHSKALIENVLDLTPVVDLGPDVFTNTRPLWHPPGARGIYGGAAIAQSLSAAMRTVPADYAVHSMHCYFVLAGDSEIPILYHVERVRDGRSFVTRTVQARQRGRPIFTTTLSFSRVGSGGEKTLHHAVSKPDVPLPEEAEPGSLKALSNAGGGPFESRKAGILNRTSPNPEDKKVRRYIRARGAISEEGGYQAHLSALAYITDSYFIGTVSIVHDVPRFSSPAELEKLLNALKNPSDLDDEDITRALRELKEEEAAELRRRLEGALNRATGPKEVDHKEVGMMVSLDHSIYFHNPRAFRADEWMLSEIESPWAGEGRGLAIQKLWSKDGVLIATCTQEVCICFYSLYSGGQC

SEQ ID NO: 69 - protein, 525 aa, Penicillium Chrysogenum
MSASALLKSRVRRPSYLKKLAKPEDLLHHFPNGTYIGWSGFTGVGYPKMTPIALADHVEKNNLQGQLKYNLFVGASSGAETENRWARLNMIERRSPHQVGKEIAKGINNGQIKFFDKHLSMFPSDLVYGYYTLNKSKPTIDVAVIEASAITENGGIIPGASVGASPELIQMADKVIIEVNTSMPSFEGLHDITCSDLPPGRKPYLIMAPEDRIGTSYIPIDPEKVVAIVESNYPDQTLPNAPEDEGSQAIASNLIEFLKHEVNHGRLPPNLLPIQSGIGNIANAVVGGLSKGGADFKNLKVWTEVLQDSFLDLFDSGNLDFATATSIRFSPDGFKRFYDNWEQYAGKLLLRSQQVSNSPEIIRRLGCIGMNTPVEVDIYAHANSTCVMGSRMLNGLGGSADFLRNSKYSIMHTPSARPTKTDPTGVSCIVPFATHIDQTEHDLDVVVTEQGLADVRGLSPRERARVIIKNCSHPDYTPILTDYLDRAEFECLRKGMGHEPHMLFQAFNMHKNLQEKGTMKIDSWE

SEQ ID NO: 70 - protein, 253 aa, Penicillium Chrysogenum
MDKYTIPLEKAVELTPIPSEPDTFTNAQPLWSFAGGYGVYGGSTVAHCLVAAQKTVPCDYVAHSLHCGFVSPGNPKRPIEYRVERTRDGKSFITRTVHATQKAGVISEAIVNFVRVGTYSNNASHDLVNTQIRYWVRAKDPIQQRSPQAQLAALAYMSDAYLIGAAVQVHDVAGQAFGTKMAMAASLNHTIYFHNPEAVRADEWMCSERESPWAGNDRALVVQRVWSPEGILVATCVQEGVLRVQVPSEKVKL

SEQ ID NO: 71 - protein, 462 aa, Penicillium Chrysogenum
MFGLSRRSALARSKSLAALPARAAVAAQPSCINTQGFHSTPSQAASRPTWMPMRVKTPWIEALTQIREAQKAGPQENAGQSVKRDLSPKKMSDSYYSAILPLAQDKWLLDSYLNASGHIRLGSLLMDLDALAGIVAYRHTGDGVSTVTAACDRITIENPLMEICDLELSGQCTYATGRSSMEISLQVTKARPEGQEAKPEDILITCAFTMVSLDPATKAPVPVAPLIVETEEEKRLFQKGEANYQAKKALRTRSLLQKSPDDEESNLIHSMWTKEMSYLNPQNPATRPANQVFMSDTVLKSAMIMQPQDRNRHNFMIFGGFLLKQTFELAFCCAASFAHARPNFVALDPSTFENPVPVGSVLYLRATVSYTEPEEREGDSTKYTKVQVRVDSKVRDVEHGTKKSTGMFNYTFLVEKDVQVMPKGYGEFMLWADARRRAQNAAAIDPAHKMSALRSIKDSVTE

SEQ ID NO: 72 - protein, 357 aa, Penicillium Chrysogenum
MSPQRGAPDNDDLTSPHSFVELMSLQRLEDALITYPDSAKPEKIERFRSLATPYNPGQGTRSFGGHVYAQSAYAASKTVGPGLVIHDMTGTFILGGLLDTPYVYTVRHIRDGYMYSTRAVDARQAGRICFSCICSFKRDEKQRLFQHQPASAQARFDSILSAKRPEDQEPSPSVDAEWWIEAVRQGNISESEFPGLDVRKTDMKDYNCAEDVKQHPERYRQLTQYRLKGSPEEDPAASLAQIREREENGEYDNLYACAHMYSSDKNSLLLIPRALGIKNWTEMASLTLTVIVHQHGEALRMVNWDSIGDSDVGVDKLPMKWFVQEGWTPRATENRGTHESHLWSPDGTLLATSLQDN

SEQ ID NO: 73 - protein, 320 aa, Mus musculus
MSAPEGLGDAHGDADRGDLSGDLRSVLVTSVLNLEPLDEDLYRGRHYWVPTSQRLFGGQIMGQALVAAAKSVSEDVHVHSLHCYFVRAGDPKVPVLYHVERIRTGASFSVRAVKAVQHGKAIFICQASFQQMQPSPLQHQFSMPSVPPPEDLLDHEALIDQYLRDPNLHKKYRVGLNRVAAQEVPIEIKVVNPPTLTQLQALEPKQMFWVRARGYIGEGDIKMHCCVAAYISDYAFLGTALLPHQSKYKVNFMASLDHSMWFHAPFRADHWMLYECESPWAGGFRGLVHGRLWRRDGVLAVTCAQEGVIRLKPQVSESKL

SEQ ID NO: 74 - protein, 472 aa, Clostridium kluyveri
MSNEVSIKELIEKAKAAQKKLEAYSQEQVDVLVKALGKVVYDNAEMFAKEAVEETEMGVYEDKVAKCHLKSGAIWNHIKDKKTVGIIKEEPERALVYVAKPKGVVAATTPITNPVVTPMCNAMAAIKGRNTIIVAPHPKAKKVSAHTVELMNAELKKLGAPENIIQIVEAPSREAAKELMESADVVIATGGAGRVKAAYSSGRPAYGVGPGNSQVIVDKGYDYNKAAQDIITGRKYDNGIICSSEQSVIAPAEDYDKVIAAFVENGAFYVEDEETVEKFRSTLFKDGKINSKIIGKSVQIIADLAGVKVPEGTKVIVLKGKGAGEKDVLCKEKMCPVLVALKYDTFEEAVEIAMANYMYEGAGHTAGIHSDNDENIRYARTVLPISRLVVNQPATTAGGTVLPISRLVVNQPATTAGGSFNNGFNPTTTLGCGSWGRNSISENLTYEHLINVSRIGYFNKEAKVPSYEEIWG

SEQ ID NO: 75 - protein, 451 aa, Porphyromonas gingivalis
MEIKEMVSLARKAQKEYQATHNQEAVDNICRAAAKVIYENAAILAREAVDETGMGVYEHKVAKNQGKSKGVWYNLHNKKSIGILNIDERTGMIEIAKPIGVVGAVTPTTNPIVTPMSNIIFALKTCNAIIIAPHPRSKKCSAHAVRLIKEAIAPFNVPEGMVQIIEEPSIEKTQELMGAVDVVVATGGMGMVKSAYSSGKPSFGVGAGNVQVIVDSNIDFEAAAEKIITGRAFDNGIICSGEQSIIYNEADKEAVFTAFRNHGAYFCDEAEGDRARAAIFENGAIAKDVVGQSVAFIAKKANINIPEGTRILVVEARGVGAEDVICKEKMCPVMCALSYKHFEEGVEIARTNLANEGNGHTCAIHSNNQAHIILAGSELTVSRIVVNAPSATTAGGHIQNGLAVTNTLGCGSWGNNSISENFTYKHLLNISRIAPLNSSIHIPDDKEIWEL

SEQ ID NO: 76 - protein, 876 aa, Clostridium kluyveri
MKVTNVEELMKKLQKVRQAQEKFSTYTQEQVDEIFKQAAMAANSARIKLAKMAVEETGMGIVEDKVIKNHFVSEYVYNKYKDEQTCGVLERDEGFGMVRIAEPVGVIAAVVPTTNPTSTAIFKALIALKTRNGIVFSPHPRAKRSTVAAAKIVLDAAVEAGAPVEIIGWIDEPSIELSQLVMKEADLILATGGPGMVRAAYSSGKPAIGVGPGNTPVIIDDSANIKMAVNSILLSKSFDHGVICASEQSVMVLDRIYEEVKTEFSERGGYILKNDEIDKVRETILVNGSISPDIVGQSARKIAEMAGVKVPERTKILIGEVESVELEEPFSREKLSPVLAMYRVKNFNDGLKKAARLVELGGIGHTSVLYVNTMTQKEKVEKFSEAMKTGRTLINMPSAQGAIGDLYNFKLAPSLTLGCGSWGGNSISENVGPKHLLNIKSIAERRENMLWFRVPEKIYFKYGALGTALKELKTMHKKKVFIVTDKVLYQLGYTDSITKILGEMGVGYKIFTDVEPDPTLATAKKGSAEMLQYNPDTIISVGGGSAMDAAKIMWVMYEHPEIKFEDLAMRFMDIRKRVYTFPKMGEKSMMISVATSAGTGSEVTPFTVITDEKTGAKYPLADYELTPDIAIIDAELMMNMPKGLTAASGIDAMTHALESYVSVMASEYTNGLALEAIRLIFKYLPLAYAEGTTNVKAREKMAHASTMAGMAFANAFLGVCHSMAHKLGAAHHIPHGIANALMIDEVIKFNAVNDPRKQAIFPQYKYPNAKWRYARIADYLELGGNSEDEKVGLLIKAIDELKEKINIPKTIREAGVAEKKFYATLDDMSEQAFDDQCTGANPRYPLISEIKQMYINAFDKVSPVVDEEEKLKVSLL

SEQ ID NO: 77 - protein, 491 aa, Clostridium kluyveri
MEIMDKDLQSIQEVRTLIAKAKKAQAEFKNFSQEAVNKVIEKIAKATEVEAVKLAKLAYEDTGYGKWEDKVIKNKFSSIVVYNYIKDLKTVGILKEDKEKKLIDIAVPLGVIAGLIPSTNPTSTAIFKVLIALKAGNAIVFSPHPTAVRSITETVKIMQKAAVEAGAPDGLIQCMSILTVEGTAELMKNKDTALILATGGEGMVRAAYSSGTPAIGVGPGNGPCFIERTADIPTAVRKVIGSDTFDNGVICASEQSIIAETVKKAEIIEEFKRQKGYFLNAEESEKVGKILLRANGTPNPAIVGKDVQALAKLAGISIPSDAVILLSEQTDVSPKNPYAKEKLAPVLAFYTVEDWHEACEKSLALLHNQGSGHTLIIHSQNEEIIREFALKKPVSRILVNSPGSLGGIGGATNLVPSLTLGCGAVGGSATSDNVGPENLFNIRKVAYGTTTVEEIREAFGVGAASSSAPAEPEDNEDVQAIVKAIMAKLNL

SEQ ID NO: 78 - protein, 491 aa, Clostridium kluyveri; identical to SEQ ID NO: 77

SEQ ID NO: 79 - protein, 469 aa, Propionibacterium freudenreichi
MTISPELIQQVVRETVREVISRQDSGTDAPSGTDGIFTDMNSAVDAADVAWRQYMDCSLRDRNRFIQAIRDVASEPDNLEYMATATVEETGMGNVPHKILKNRYAALYTPGTEDIITEAWSGDDGLTTVEFSPFGVIGAITPTTNPTETVINNTIGMLAAGNAVVFSPHPRAKKITLWLVRKINRALAAAGAPANLVVTVEEPSIDNTNAMMSHEKVRMLVATGGPGIVKAVLSSGKKAIGAGAGNPPAVVDDTADIAKAARDIVDGASFDNNLPCTAEKEVLAVDSIADLLKFEMLKHGCFELKDRAVMDKLAALVTKGQHANAAYVGKPAAQLASEVGLSAPKDTRLLICEVPFDHPFVQVELMMPILPIVRMPDVDTAIDKAVEVEHGNRHTAVMHSSNVNALTKMGKLIQTTIFVKNGPSYNGIGIDGEGFPTFTIAGPTGEGLTSARCFARKRRCVLKSGLNIR

SEQ ID NO: 80 - protein, 858 aa, Clostridium acetobutylicum
MKVTNQKELKQKLNELREAQKKFATYTQEQVDKIFKQCAIAAAKERINLAKLAVEETGIGLVEDKIIKNHFAAEYIYNKYKNEKTCGIIDHDDSLGITKVAEPIGIVAAIVPTTNPTSTAIFKSLISLKTRNAIFFSPHPRAKKSTIAAAKLILDAAVKAGAPKNIIGWIDEPSIELSQDLMSEADIILATGGPSMVKAAYSSGKPAIGVGAGNTPAIIDESADIDMAVSSIILSKTYDNGVICASEQSILVMNSIYEKVKEEFVKRGSYILNQNEIAKIKETMFKNGAINADIVGKSAYIIAKMAGIEVPQTTKILIGEVQSVEKSELFSHEKLSPVLAMYKVKDFDEALKKAQRLIELGGSGHTSSLYIDSQNNKDKVKEFGLAMKTSRTFINMPSSQGASGDLYNFAIAPSFTLGCGTWGGNSVSQNVEPKHLLNIKSVAERRENMLWFKVPQKIYFKYGCLRFALKELKDMNKKRAFIVTDKDLFKLGYVNKITKVLDEIDIKYSIFTDIKSDPTIDSVKKGAKEMLNFEPDTIISIGGGSPMDAAKVMHLLYEYPEAEIENLAINFMDIRKRICNFPKLGTKAISVAIPTTAGTGSEATPFAVITNDETGMKYPLTSYELTPNMAIIDTELMLNMPRKLTAATGIDALVHAIEAYVSVMATDYTDELALRAIKMIFKYLPRAYKNGTNDIEAREKMAHASNIAGMAFANAFLGVCHSMAHKLGAMHHVPHGIACAVLIEEVIKYNATDCPTKQTAFPQYKSPNAKRKYAEIAEYLNLKGTSDTEKVTALIEAISKLKIDLSIPQNISAAGINKKDFYNTLDKMSELAFDDQCTTANPRYPLISELKDIYIKSF

SEQ ID NO: 81 - protein, 862 aa, Clostridium acetobutylicum
MKVTTVKELDEKLKVIKEAQKKFSCYSQEMVDEIFRNAAMAAIDARIELAKAAVLETGMGLVEDKVIKNHFAGEYIYNKYKDEKTCGIIERNEPYGITKIAEPIGVVAAIIPVTNPTSTTIFKSLISLKTRNGIFFSPHPRAKKSTILAAKTILDAAVKSGAPENIIGWIDEPSIELTQYLMQKADITLATGGPSLVKSAYSSGKPAIGVGPGNTPVIIDESAHIKMAVSSIILSKTYDNGVICASEQSVIVLKSIYNKVKDEFQERGAYIIKKNELDKVREVIFKDGSVNPKIVGQSAYTIAAMAGIKVPKTTRILIGEVTSLGEEEPFAHEKLSPVLAMYEADNFDDALKKAVTLINLGGLGHTSGIYADEIKARDKIDRFSSAMKTVRTFVNIPTSQGASGDLYNFRIPPSFTLGCGFWGGNSVSENVGPKHLLNIKTVAERRENMLWFRVPHKVYFKFGCLQFALKDLKDLKKKRAFIVTDSDPYNLNYVDSIIKILEHLDIDFKVFNKVGREADLKTIKKATEEMSSFMPDTIIALGGTPEMSSAKLMWVLYEHPEVKFEDLAIKFMDIRKRIYTFPKLGKKAMLVAITTSAGSGSEVTPFALVTDNNTGNKYMLADYEMTPNMAIVDAELMMKMPKGLTAYSGIDALVNSIEAYTSVYASEYTNGLALEAIRLIFKYLPEAYKNGRTNEKAREKMAHASTMAGMASANAFLGLCHSMAIKLSSEHNIPSGIANALLIEEVIKFNAVDNPVKQAPCPQYKYPNTIFRYARIADYIKLGGNTDEEKVDLLINKIHELKKALNIPTSIKDAGVLEENFYSSLDRISELALDDQCTGANPRFPLTSEIKEMYINCFKKQP

SEQ ID NO: 82 - protein, 453 aa, Vibrio fluvialis
MNKPQSWEARAETYSLYGFTDMPSLHQRGTVVVTHGEGPYIVDVNGRRYLDANSGLWNMVAGFDHKGLIDAAKAQYERFPGYHAFFGRMSDQTVMLSEKLVEVSPFDSGRVFYTNSGSEANDTMVKMLWFLHAAEGKPQKRKILTRWNAYHGVTAVSASMTGKPYNSVFGLPLPGFVHLTCPHYWRYGEEGETEEQFVARLARELEETIQREGADTIAGFFAEPVMGAGGVIPPAKGYFQAILPILRKYDIPVISDEVICGFGRTGNTWGCVTYDFTPDAIISSKNLTAGFFPMGAVILGPELSKRLETAIEAIEEFPHGFTASGHPVGCAIALKAIDVVMNEGLAENVRRLAPRFEERLKHIAERPNIGEYRGIGFMWALEAVKDKASKTPFDGNLSVSERIANTCTDLGLICRPLGQSVVLCPPFILTEAQMDEMFDKLEKALDKVFAEVA

SEQ ID NO: 83 - protein, 449 aa, Bacillus weihenstephanensis
MQATEQTQSLKKTDEKYLWHAMRGAAPSPTNLIITKAEGAWVTDIDGNRYLDGMSGLWCVNVGYGRKELARAAFEQLEEMPYFPLTQSHVPAIKLAEKLNEWLDDEYVIFFSNSGSEANETAFKIARQYHQQKGDHGRYKFISRYRAYHGNSMGALAATGQAQRKYKYEPLGQGFLHVAPPDTYRNPEDVHTLASAEEIDRVMTWELSQTVAGVIMEPIITGGGILMPPDGYMGKVKEICEKHGALLICDEVICGFGRTGKPFGFMNYGVKPDIITMAKGITSAYLPLSATAVRREVYEAFVGSDDYDRFRHVNTFGGNPAACALALKNLEIMENEKLIERSKELGERLLYELEDVKEHPNVGDVRGKGLLLGIELVEDKQTKEPASIEKMNKVINACKEKGLIIGKNGDTVAGYNNILQLAPPLSITEEDFTFIVKTMKECLSRINGQ

SEQ ID NO: 84 - protein, 456 aa, Pseudomonas aeruginosa
MNSQITNAKTREWQALSRDHHLPPFTDYKQLNEKGARIITKAEGVYIWDSEGNKILDAMAGLWCVNVGYGREELVQAATRQMRELPFYNLFFQTAHPPVVELAKAIADVAPEGMNHVFFTGSGSEANDTVLRMVRHYWATKGQPQKKVVIGRWNGYHGSTVAGVSLGGMKALHEQGDFPIPGIVHIAQPYWYGEGGDMSPDEFGVWAAEQLEKKILEVGEENVAAFIAEPIQGAGGVIVPPDTYWPKIREILAKYDILFIADEVICGFGRTGEWFGSQYYGNAPDLMPIAKGLTSGYIPMGGVVVRDEIVEVLNQGGEFYHGFTYSGHPVAAAVALENIRILREEKIIEKVKAETAPYLQKRWQELADHPLVGEARGVGMVAALELVKNKKTRERFTDKGVGMLCREHCFRNGLIMRAVGDTMIISPPLVIDPSQIDELITLARKCLDQTAAAVLA

SEQ ID NO: 85 - protein, 538 aa, Penicillium Chrysogenum
MTALRISTTLSRKALTACRPRLFLGVRTSVRPWQPFSTSTSTRYSITTPLKSLAPKVERSGSKLYKDADAAVADIKSGSTILSSGFGLCGVAETLINAMHRRGADQLHSLTAVSNNAGAAGKGGLSTLSQNGQINRLILSYLGNNKALEKKYLTGHIAIELCPQGTLAERLRAGGAGIPAFFTPTGEGKIPVRMDESGKVLESGKPRETREFNGKTYLMEEALTGDVAILRAWKADEAGNCVFRYTTKAFGPIMAKAATLTIVEAENIVPIGSIDPNDVDLPGIFVDRIVPATDDKHIEIRKLRSGETTVAGSGKDEARIQRELIGRRAAKELKPGFYVNLGVGIPTLAPSFLPKDVKVWIQSENGILGMGDYPTEQELDPDIINAGKETVTLVPGAATFDSSESFGMIRGGHVDVSILGALQVSANGDLANYMIPGKVFKGMGGAMDLISNPEKTKIVVATSHVAKDGSPKIVQKCSLPLTGANVVSTIITDLCVFQVDRATGELTLTELAPGVEVEEVQSKTDAKFTIADTLEIME

SEQ ID NO: 86 - DNA, 1362 bp, vibrio fluvialis
  CDS (1)..(1362)
atgaacaaaccgcaaagctgggaagcccgggccgagacctattcgctctatggtttcaccgacatgccttcgctgcatcagcgcggcacggtcgtcgtgacccatggcgagggaccctatatcgtcgatgtgaatggccggcgttatctggacgccaactcgggcctgtggaacatggtcgcgggctttgaccacaaggggctgatcgacgccgccaaggcccaatacgagcgttttcccggttatcacgcctttttcggccgcatgtccgatcagacggtaatgctgtcggaaaagctggtcgaggtgtcgccctttgattcgggccgggtgttctatacaaactcggggtccgaggcgaatgacaccatggtcaagatgctatggttcctgcatgcagccgagggcaaaccgcaaaagcgcaagatcctgacccgctggaacgcctatcacggcgtgaccgccgtttcggccagcatgaccggcaagccctataattcggtctttggcctgccgctgccgggctttgtgcatctgacctgcccgcattactggcgctatggcgaagagggcgaaaccgaagagcagttcgtcgcccgcctcgcccgcgagctggaggaaacgatccagcgcgagggcgccgacaccatcgccggtttctttgccgaaccggtgatgggcgcgggcggcgtgattcccccggccaagggctatttccaggcgatcctgccaatcctgcgcaaatatgacatcccggtcatctcggacgaggtgatctgcggtttcggacgcaccggtaacacctggggctgcgtgacctatgactttacacccgatgcaatcatctcgtccaagaatcttacagcgggctttttccccatgggggcggtgatccttggcccggaactttccaaacggctggaaaccgcaatcgaggcgatcgaggaattcccccatggctttaccgcctcgggccatccggtcggctgtgctattgcgctgaaagcaatcgacgtggtgatgaatgaagggctggctgagaacgtccgccgccttgccccccgtttcgaggaaaggctgaaacatatcgccgagcgcccgaacatcggtgaatatcgcggcatcggcttcatgtgggcgctggaggctgtcaaggacaaggcaagcaagacgccgttcgacggcaacctgtcggtcagcgagcgtatcgccaatacctgcaccgatctggggctgatttgccggccgcttggtcagtccgtcgtcctttgtccgccctttatcctgaccgaggcgcagatggatgagatgttcgataaactcgaaaaagcccttgataaggtctttgccgaggttgcctga

SEQ ID NO: 87 - protein, 453 aa, vibrio fluvialis; identical to SEQ ID NO: 82

SEQ ID NO: 88 - DNA, 1362 bp, Artificial
  Vibrio fluvialis JS17 omega-aminotransferase codon optimised gene
atgaataaaccacagtcttgggaagctcgtgctgaaacctatagcctgtacggctttaccgatatgccgtctctgcaccagcgtggtactgtagtggtaacgcacggtgagggcccgtacatcgtggacgttaatggccgccgttacctggatgcaaacagcggcctgtggaacatggttgcgggcttcgaccacaaaggcctgatcgatgccgcaaaagcgcagtacgaacgcttcccgggttatcacgcgttctttggccgtatgagcgaccagactgtgatgctgagcgaaaaactggttgaagtgtccccgttcgatagcggtcgtgtcttttacactaactctggcagcgaggctaacgataccatggttaagatgctgtggttcctgcacgcagcggaaggcaaacctcagaaacgtaaaattctgacccgttggaacgcttatcacggtgtgactgctgtttccgcatctatgaccggtaaaccgtataacagcgtgttcggtctgccgctgcctggcttcgtgcatctgacctgcccgcactactggcgttatggtgaggaaggcgaaactgaggaacagttcgtggcgcgtctggctcgtgaactggaagaaaccattcaacgcgaaggtgcagatactatcgcgggcttctttgcggagcctgttatgggtgccggcggtgtgattccgccggcgaagggctatttccaggcaatcctgccgatcctgcgcaagtacgacattccggttatttctgacgaagtgatctgcggcttcggccgcaccggtaacacctggggctgcgtgacgtatgacttcactccggacgcaatcattagctctaaaaacctgactgcgggtttcttccctatgggcgccgtaatcctgggcccagaactgtctaagcgcctggaaaccgccatcgaggcaatcgaagagttcccgcacggtttcactgctagcggccatccggtaggctgcgcaatcgcgctgaaggcgatcgatgttgtcatgaacgagggcctggcggaaaacgtgcgccgcctggcgccgcgttttgaagaacgtctgaaacacattgctgagcgcccgaacattggcgaatatcgcggcatcggtttcatgtgggccctggaagcagttaaagataaagctagcaagaccccgttcgacggcaacctgtccgtgagcgaacgtatcgctaatacctgtacggacctgggtctgatctgccgtccgctgggtcagtccgtagttctgtgcccaccatttatcctgaccgaagcgcagatggatgaaatgttcgataaactggagaaagctctggataaagtgttcgctgaagtcgcgtaa

SEQ ID NO: 89 - DNA, 1350 bp, Bacillus weihenstephanensis
  CDS (1)..(1350)
gtgcaagcgacggagcaaacacaaagtttgaaaaaaacagatgaaaagtacctttggcatgcgatgagaggagcagcccctagtccaacgaatttaattatcacaaaagcagaaggggcatgggtgacggatattgatggaaaccgttatttagacggtatgtccggtctttggtgcgtgaatgttgggtatggtcgaaaagaacttgcaagagcggcgtttgaacagcttgaagaaatgccgtatttccctctgactcaaagtcatgttcctgctattaaattagcagaaaaattgaatgaatggcttgatgatgaatacgtcattttcttttctaacagtggatcggaagcgaatgaaacagcatttaaaattgctcgtcaatatcatcaacaaaaaggtgatcatggacgctataagtttatttcccgctaccgcgcttatcacggtaactcaatgggagctcttgcagcaacaggtcaagcacagcgaaagtataaatatgaaccactcgggcaaggattcctgcatgtagcaccgcctgatacgtatcgaaatccagaggatgttcatacactggcaagtgctgaggaaatcgatcgtgtcatgacatgggagttaagccaaacagtagccggtgtgattatggagccaatcattactgggggcggaattttaatgcctcctgatggatatatgggaaaagtaaaagaaatttgcgagaagcacggtgcgttgctcatttgtgatgaagttatatgtggatttggccggacagggaagccatttggatttatgaattatggcgtcaaaccagatatcattacaatggcaaaaggtattacaagtgcgtatcttcctttgtcagcaacagcagttagacgagaggtttatgaggcattcgtaggtagtgatgattatgatcgcttccgccatgtaaatacgttcggagggaatcctgctgcttgcgctttagctttgaagaatttagaaattatggagaatgagaaactcattgaacgttccaaagaattgggtgaacgactgttatatgagctagaggatgtaaaagagcatccaaacgtaggggatgttcgcggaaagggccttcttttaggcattgaactagtggaagataagcaaacaaaagaaccggcttccattgaaaagatgaacaaagtcatcaatgcttgtaaagaaaaaggtctaattattggtaaaaatggtgacactgtcgcaggttacaataatattttgcagcttgcacctccattaagcatcacagaggaagactttacttttatcgttaaaacaatgaaagaatgtttatcccgcattaacgggcagtaa

SEQ ID NO: 90 - protein, 449 aa, Bacillus weihenstephanensis
VQATEQTQSLKKTDEKYLWHAMRGAAPSPTNLIITKAEGAWVTDIDGNRYLDGMSGLWCVNVGYGRKELARAAFEQLEEMPYFPLTQSHVPAIKLAEKLNEWLDDEYVIFFSNSGSEANETAFKIARQYHQQKGDHGRYKFISRYRAYHGNSMGALAATGQAQRKYKYEPLGQGFLHVAPPDTYRNPEDVHTLASAEEIDRVMTWELSQTVAGVIMEPIITGGGILMPPDGYMGKVKEICEKHGALLICDEVICGFGRTGKPFGFMNYGVKPDIITMAKGITSAYLPLSATAVRREVYEAFVGSDDYDRFRHVNTFGGNPAACALALKNLEIMENEKLIERSKELGERLLYELEDVKEHPNVGDVRGKGLLLGIELVEDKQTKEPASIEKMNKVINACKEKGLIIGKNGDTVAGYNNILQLAPPLSITEEDFTFIVKTMKECLSRINGQ

SEQ ID NO: 91 - DNA, 1350 bp, Artificial
  B. weihenstephanensis KBAB4 aminotransferase codon-optimised gene
atgcaggctaccgaacaaacccaatctctgaaaaagactgacgaaaaatatctgtggcacgcgatgcgcggtgcagctccgtctccgaccaacctgattattaccaaagctgaaggcgcgtgggtgaccgacattgacggtaaccgttatctggatggcatgagcggcctgtggtgtgttaatgtcggttatggccgtaaggagctggcgcgcgcggcatttgaacaactggaagaaatgccgtacttcccgctgactcaaagccatgtgccggctatcaaactggcggaaaaactgaacgaatggctggacgacgaatacgtgattttcttctctaattctggctccgaagcaaacgaaaccgcattcaaaatcgcccgtcaatatcaccagcagaaaggtgaccacggccgctataaattcatcagccgttatcgtgcataccatggtaattctatgggtgcgctggctgctaccggtcaggctcagcgcaaatacaagtacgaaccgctgggtcagggttttctgcacgttgcaccaccggatacctaccgtaacccggaagacgtccacaccctggcttctgccgaagaaatcgatcgtgttatgacctgggagctgtcccagactgttgcgggtgttatcatggaacctattattaccggtggtggcattctgatgccgccggacggttatatgggtaaagtcaaggaaatctgcgaaaaacacggcgcgctgctgatctgcgatgaagttatctgtggcttcggtcgcaccggcaaaccatttggcttcatgaattatggcgtaaaacctgacattattaccatggctaaaggcattacttccgcttatctgccgctgagcgcgaccgcagttcgccgcgaagtttatgaagcgtttgttggttctgatgattacgaccgtttccgtcatgtaaacacgtttggcggtaacccagcggcatgtgcgctggcgctgaaaaacctggaaatcatggaaaacgaaaagctgatcgaacgtagcaaagaactgggtgaacgtctgctgtacgaactggaagatgtcaaagaacacccgaacgtgggcgatgttcgcggtaaaggcctgctgctgggtattgaactggttgaagacaaacagaccaaggaaccggcttccattgaaaagatgaacaaagtgattaacgcgtgcaaagagaaaggcctgatcattggtaagaacggtgataccgtggcaggttataacaacattctgcagctggcgccgcctctgagcatcactgaagaagatttcaccttcatcgtcaaaactatgaaggagtgcctgagccgcatcaatggtcagtaa

SEQ ID NO: 92 - protein, 255 aa, Saccharomyces cerevisiae; Hydroxyacyl-thioester dehydratase type 2, mitochondrial (P38790)
MAELRVLVAVKRVIDYAVKIRVKPDRTGVVTDGVKHSMNPFCEIAVEEAVRLKEKKLVKEVIAVSCGPAQCQETIRTALAMGADRGIHVEVPPAEAERLGPLQVARVLAKLAEKEKVDLVLLGKQAIDDDCNQTGQMTAGFLDWPQGTFASQVTLEGDKLKVEREIDGGLETLRLKLPAVVTADLRLNEPRYATLPNIMKAKKKKIEVIKPGDLGVDLTSKLSVISVEDPPQRTAGVKVETTEDLVAKLKEIGRI

SEQ ID NO: 93 - DNA, 860 bp, artificial
  Microscilla marina ATCC 23134 Peroxisomal trans-2-enoyl-CoA reductase;  EC=1.3.1.38 (A1ZFB1)
ggtaccggatccctaacaggaggaattaaccatggtccagaaagacctgttcaaagacaaagttgttctggtaactggcggtcgttctggtatcggttacgcaatttctcagatgatgctggaactgggtgcgaaagttgttatcgcttctcgcaaagaggatctgctgaaacaggctgctgaagaactgtctcagtacggtgaatgctcctacctggcttgcgacatccgtgaatctgaccagcgtactgcgctgatggagaagatcaaagctgacaacggtcgtctggatatcctggttaacaacgctggcggtcagttcccggcaccggcagaaaccatctctgaaaacggctgggacgctgttatcaacaacaacctgaacggtactttccacatgtcctctctgatggcgcgtcacttcttcatcccgcagaaagaaggttgcatcatcaacatcatcgctaacatctaccgcggtttcccgtctatggttcacaccggtgcagcacgtgctggcgttgaaaacctgaccaaaactctggcggttgagtggggcgactacaacatccgcgttaacgcgattgctccgggtactatcgaatcttccggtctggatacttacccgaagccggtacaggacatcctgggtgaagcgcgtgctgcagtaccactgaaacgcttcggtactgttactgaaatcgctaacaccacttgcttcctggcttctccgctggcttcttacatctccggtgtttctctgtacgttgacggtgcacagcacctgaacggtggtgacccgatgaagctgactcgcctgatgcgtgcattcaccaagtctcgtgagctctaataagctt

SEQ ID NO: 94 - protein, 273 aa, Microscilla marina ATCC 23134 Peroxisomal trans-2-enoyl-CoA reductase;  EC=1.3.1.38 (A1ZFB1)
MVQKDLFKDKVVLVTGGRSGIGYAISQMMLELGAKVVIASRKEDLLKQAAEELSQYGECSYLACDIRESDQRTALMEKIKADNGRLDILVNNAGGQFPAPAETISENGWDAVINNNLNGTFHMSSLMARHFFIPQKEGCIINIIANIYRGFPSMVHTGAARAGVENLTKTLAVEWGDYNIRVNAIAPGTIESSGLDTYPKPVQDILGEARAAVPLKRFGTVTEIANTTCFLASPLASYISGVSLYVDGAQHLNGGDPMKLTRLMRAFTKSRET

SEQ ID NO: 95 - DNA, 1241 bp, Artificial
  Clostridium beijerinckii (strain ATCC 51743 / NCIMB 8052), Putative reductase Cbei_2086;  EC=1.3.1 (A6LV73)
ggtaccggatccctaacaggaggaattaatcatgatcttcaagccggaactgatcaaaggtatcgctaaaacttctcacccgtacggttgccgtaaagaagttctgaaccagatcgaatactgcaaaaacgctaagcagttccacggtccgaagaaagttctgatcatcggtgcttcttccggtttcggtctggcaactcgcatttctctggcgttcggtggtgcgaaagcagacaccatcggtgtttctttcgaaaccggtatcactgaccgccgtactggtactgcaggctggtacaacaacatcttcttcaaagagttcgcagaaaaagaaggtctgattgctaaaaacttcatcggtgacgcattctctgacgaagttaaagaaaacgttatcaaatacatcaaaaacgagttcggtaagatcgatctgctgatctactctctggcttctccgcgccgtaaagatccgaaaaccggtaacatctacgactccactctgaaaaccacttctggcgagttccagggcccaaccatcgacatggaaactgacgaactggttactaccaaagttaactccgcaactgacaaagaaatcgaagcgaccaagaaagtaatgggtggtgaagattggtctgaatggtgcaaactgctgctggaaaacgactgcctgtctgacaaagctatcactatctcttactcttacatcggtgcttctcgcacttacaaaatctaccgtgaaggtactatcggtgaagcgaagcgtcacctggaaaacactgcgattcagatcgacaaagaatggcagaagaagatcaacggtaaagcattcgtttctgttaacaaagcaatcgttaccaaggcttctgcttacatcccgtctttctctctgtacgctgctgttctgtacaaagtaatgaaagaaaaaaatctgcacgaaaactgcatcatgcagatgcagcgtatgttcgctgacaaaatctacgctgaaaatctgctggagttcgacgactccggtcgtctgcgtatggacgactgggaactgcgtgaagatgtacagtctgaagttaacgaactgtgggaaaaaatcactccggataacttcaagatcctgtctgactacgacggttacaagaaagagttcatgcagctgaacggcttcgaaatcgacggtgttaactactctgaagatatcgacatcgaagcgctgaagcgcctggaaccggagctctaataagctt

SEQ ID NO: 96 - protein, 400 aa, Clostridium beijerinckii (strain ATCC 51743 / NCIMB 8052), Putative reductase Cbei_2086;  EC=1.3.1 (A6LV73)
MIFKPELIKGIAKTSHPYGCRKEVLNQIEYCKNAKQFHGPKKVLIIGASSGFGLATRISLAFGGAKADTIGVSFETGITDRRTGTAGWYNNIFFKEFAEKEGLIAKNFIGDAFSDEVKENVIKYIKNEFGKIDLLIYSLASPRRKDPKTGNIYDSTLKTTSGEFQGPTIDMETDELVTTKVNSATDKEIEATKKVMGGEDWSEWCKLLLENDCLSDKAITISYSYIGASRTYKIYREGTIGEAKRHLENTAIQIDKEWQKKINGKAFVSVNKAIVTKASAYIPSFSLYAAVLYKVMKEKNLHENCIMQMQRMFADKIYAENLLEFDDSGRLRMDDWELREDVQSEVNELWEKITPDNFKILSDYDGYKKEFMQLNGFEIDGVNYSEDIDIEALKRLEPET

SEQ ID NO: 97 - DNA, 1238 bp, Artificial
  Aeromonas hydrophila subsp. hydrophila (strain ATCC 7966 / NCIB 9240), Trans-2-enoyl-CoA reductase;  EC=1.3.1.44 (A0KLI7)
ggtaccggatccctaacaggaggaattaatcatgatcatcaagccgaaagttcgtggcttcatctgcaccactactcacccggttggttgcgaagctaacgttcgtcgtcagatcgcttacaccaaagcgaaaggtactatcgaaaacggtccgaagaaagttctggttatcggtgcttctaccggttacggtctggcttctcgcattgctgctgcattcggttctggtgcggcaactctgggcgtattcttcgaaaaagcgggttctgaaaccaaaactgcaactgctggctggtacaactccgcagcattcgacaaagcagctaaagaagcgggtctgtacgctaaatctatcaacggtgacgcattctctaacgaatgccgcgctaaagttatcgaactgatcaagcaggacctgggtcagatcgacctggttgtttactctctggcttctccggtacgtaagctgccggataccggtgaagttgttcgttctgcactgaaaccgatcggtgaagtttacaccactactgctatcgacaccaacaaagaccagatcatcactgcaaccgttgagccggctaacgaagaagaaatccagaacaccatcaccgtaatgggtggtcaggactgggaactgtggatggctgcgctgcgcgatgctggcgtactggcagacggtgcgaagtctgttgcttactcttacatcggtactgacctgacctggccaatctactggcacggtactctgggtcgtgcgaaagaagatttggaccgcgctgcagctgctatccgcggtgacctggcaggcaaaggtggtactgcgcacgttgctgtactgaaatctgttgttactcaggcttcttctgcgattccggtaatgccgctgtacatctctatggcattcaagattatgaaagagaaaggtatccacgaaggttgcatggaacaggttgaccgtatgatgcgtactcgtctgtacgctgcagacatggcgctggatgaccaggcgcgtatccgtatggacgactgggaactgcgtgaagatgttcagcagacttgccgcgacctgtggccgtctatcacttctgaaaacctgtgcgaactgactgactacaccggttacaagcaggagttcctgcgtctgttcggtttcggtctggaagaagttgactacgacgctgacgttaacccggacgttaagttcgacgttgttgaactagagctctaataagctt

SEQ ID NO: 98 - protein, 399 aa, Aeromonas hydrophila subsp. hydrophila (strain ATCC 7966 / NCIB 9240), Trans-2-enoyl-CoA reductase;  EC=1.3.1.44 (A0KLI7)
MIIKPKVRGFICTTTHPVGCEANVRRQIAYTKAKGTIENGPKKVLVIGASTGYGLASRIAAAFGSGAATLGVFFEKAGSETKTATAGWYNSAAFDKAAKEAGLYAKSINGDAFSNECRAKVIELIKQDLGQIDLVVYSLASPVRKLPDTGEVVRSALKPIGEVYTTTAIDTNKDQIITATVEPANEEEIQNTITVMGGQDWELWMAALRDAGVLADGAKSVAYSYIGTDLTWPIYWHGTLGRAKEDLDRAAAAIRGDLAGKGGTAHVAVLKSVVTQASSAIPVMPLYISMAFKIMKEKGIHEGCMEQVDRMMRTRLYAADMALDDQARIRMDDWELREDVQQTCRDLWPSITSENLCELTDYTGYKQEFLRLFGFGLEEVDYDADVNPDVKFDVVELET

SEQ ID NO: 99 - DNA, 1142 bp, Artificial
  Yarrowia lipolytica, Probable trans-2-enoyl-CoA reductase, mitochondrial;  EC=1.3.1.38, (Q6CBE4)
ggtaccggatccctaacaggaggaattaaccatggccggcttcggtactccgtctttcggtctgcgcttcaactccgttggtcgtgcattcgtattctctcagactggcgaaccgaaagacgttattcaggtactggaatacccaatcgaaaaaccgctggaaaaccaggttctgctgaaatctctgggcttcactatcaacccggctgacatcaaccagctggaaggtgtttacccgtctgtaccgccgaaatctgtacagatcaacaacgaagatgctgctatcggtggtaacgaaggtctgttccaggttctggacccgggtgctaaatctggtctgaagaaaggcgactgggtactgccgcgtaaaacttgcttcggcacctggcgttctcacgcgctggttgaagctgataccgttgttaagatcgacaacaccgacctgaccaaagttcaggcaactaccgtttctgttaacccgtctactgcttacgaaatgctgaaagacctgaaagaaggtgactggttcatccagaacggtggtaactccggtgttggtcgtgctgcgattcagatcggtcacatccgcggtctgaaatctatctccgttgttcgtgaccgtccggatctggaagttctgaagaaagaactgactgacctgggtgcaactcacgttatcactgaagaagaagcgtctgacaaactgttctccaagcagatcaaatcctggactggcggtaaaatcaagctggcactgaactgcatcggtggtaaatctgcaacttccatcatgcgtcagctgggtgctggcggttctatcgttacttacggtggtatgtccaagaagccgctgactttcccgactggtccgttcatcttcaaagacatcactgcgaaaggttactggctgactcgctgggctgacaagcacccggaagaaaaagcgaaaactatcgaaaacatcttcaaattctaccgcgagaagaaattcgttgctccgccagttaacatctccactctggacttctctaaaggtaacgacgttgttctgtctgagttcctggatgcactgggtaaagcacagaaaggtggtggtaagaagcagctggtacagtgggttgaatacgagctctaataagctt

SEQ ID NO: 100 - protein, 367 aa, Yarrowia lipolytica, Probable trans-2-enoyl-CoA reductase, mitochondrial;  EC=1.3.1.38, (Q6CBE4)
MAGFGTPSFGLRFNSVGRAFVFSQTGEPKDVIQVLEYPIEKPLENQVLLKSLGFTINPADINQLEGVYPSVPPKSVQINNEDAAIGGNEGLFQVLDPGAKSGLKKGDWVLPRKTCFGTWRSHALVEADTVVKIDNTDLTKVQATTVSVNPSTAYEMLKDLKEGDWFIQNGGNSGVGRAAIQIGHIRGLKSISVVRDRPDLEVLKKELTDLGATHVITEEEASDKLFSKQIKSWTGGKIKLALNCIGGKSATSIMRQLGAGGSIVTYGGMSKKPLTFPTGPFIFKDITAKGYWLTRWADKHPEEKAKTIENIFKFYREKKFVAPPVNISTLDFSKGNDVVLSEFLDALGKAQKGGGKKQLVQWVEYET

SEQ ID NO: 101 - DNA, 1856 bp, Artificial
  Clostridium kluyveri (strain ATCC 8527 / DSM 555 / NCIMB 10680) (A5N5C9)
ggtaccggatccctaacaggaggaattaaccatggacctggcagaatacaaaggcgtatgggtattcgctgaacagcgtgacggtgaactgcagaaagttgcgctgcagctggttggtaaaggtcgtgaactggctgacactctgggtgttgaactgactgcggtactgctgggttctgaagttgatgacctggcgaaagaactggttgcttacggcgcagacaacgtactgtacgcagactctccgctgctgaagcactacaccactgacggttacaccaaagttatcgacgaactgatcaaagagcgtaagccggaaatcctgctgatcggtgcgactttcatcggtcgtgacctgggtccgcgcgttgctggtcgcgtattcaccggtctgactgcagactgcaccggtctggatatcgacgaagcgaccaagaacctgatgatgactcgtccggcattcggtggtaacctgatggcaactatcgcttgcgaaaaaactcgtccgcagatgtccaccgttcgtccgggcgtattcaacgcactgccgcgcgacgcttcccgtactggtaagatcgaaaaaatcgctgctaacgttgctaaagacgacatccgtatcgaagttctggaagttgttaagtctgctggcgacaccatcgacatctctgaagcagacgttatcgtttctggtggtcgcggtctgggtggtccggacggcttcaaagttctgaaagaactggctgatctgctgggtggtactatcggtggttctcgcgctaccatcgacgctggctggatcgacaagtcttaccaggttggtcagactggtaaaaccgttcgtccgggtctgtacatcgcttgcggtatctccggtcagattcagcacctggcaggcatgcaggattccggcttcatcgttgctatcaacaaagacgaaaacgcaccgatgatgcaagttgctgatctggcgattgttggtgacctgtacaaagttgttccagagttcgttgaacaggttaaagcgctgaacttgtaataactagtctaacaggaggaattaatcatgaagatcgttgtttgcctgaaacaggttccggataccactgaagttaagatcgacccgaaaaccggtactctgatccgtgaaggcgtaccgtctatcatcaacccggatgacaaaaacgcgctggaagaatccattgctctgaaagagaaagttggcggcaccgtaactgttgtttctatgggtccgccacaggctgttgatgcgctgcgtgaagcgctggcaatgggtgctgacgaagcaatcctggtatctgaccgcgctttcgctggtgctgacactcaggcaacttcttacgcactggcaggcgcactgaaaaacctggaatacgacctgattttcgctggtcgtcaggctatcgacggtgacactgcacaggttggtccgcagatcgctgaaaaactgggtatcccgcagatcacttacgttgaaaaagttgacgttgacggtgacactctgaccgtacagcgtgcatgggaagatggttacgaagttgcgaaaatcaaaactccgtgcatgctgactgctatcaaagagctgaaccagccgcgctacatgaacatgaagaacatcttcgaagtattcaagaaagaagttaaaatctggtctgctgacgacctggacgttgacaaaaacaagctgggtctgaacggttcctgcaccaaagttaagcgttctcacaccaaagaagcgaaaggtgctggcgaaatcgttaacaagccgatcaaagaagcggttgcttactccatctccaagctgcgtgaaaaacacgttatcgagctctaataagctt

SEQ ID NO: 102 - protein, 334 aa, Clostridium kluyveri (strain ATCC 8527 / DSM 555 / NCIMB 10680) (A5N5C9)
MDLAEYKGVWVFAEQRDGELQKVALQLVGKGRELADTLGVELTAVLLGSEVDDLAKELVAYGADNVLYADSPLLKHYTTDGYTKVIDELIKERKPEILLIGATFIGRDLGPRVAGRVFTGLTADCTGLDIDEATKNLMMTRPAFGGNLMATIACEKTRPQMSTVRPGVFNALPRDASRTGKIEKIAANVAKDDIRIEVLEVVKSAGDTIDISEADVIVSGGRGLGGPDGFKVLKELADLLGGTIGGSRATIDAGWIDKSYQVGQTGKTVRPGLYIACGISGQIQHLAGMQDSGFIVAINKDENAPMMQVADLAIVGDLYKVVPEFVEQVKALNL

SEQ ID NO: 103 - protein, 259 aa, Clostridium kluyveri (strain ATCC 8527 / DSM 555 / NCIMB 10680)   (A5N5D0)
MKIVVCLKQVPDTTEVKIDPKTGTLIREGVPSIINPDDKNALEESIALKEKVGGTVTVVSMGPPQAVDALREALAMGADEAILVSDRAFAGADTQATSYALAGALKNLEYDLIFAGRQAIDGDTAQVGPQIAEKLGIPQITYVEKVDVDGDTLTVQRAWEDGYEVAKIKTPCMLTAIKELNQPRYMNMKNIFEVFKKEVKIWSADDLDVDKNKLGLNGSCTKVKRSHTKEAKGAGEIVNKPIKEAVAYSISKLREKHVI

SEQ ID NO: 104 - DNA, 1196 bp, Artificial
  Megasphaera elsdenii, Acyl-CoA dehydrogenase, short-chain specific;  EC=1.3.99.2 (Q06319)
ggtaccggatccctaacaggaggaattaaccatggacttcaacctgactgatatccagcaggacttcctgaaactggcacacgacttcggtgaaaaaaaactggcaccaaccgtaactgaacgtgaccacaaaggtatctacgacaaagagctgatcgacgaactgctgtctctgggtatcactggcgcttacttcgaagagaaatacggtggttctggtgacgacggtggtgacgttctgtcttacatcctggctgttgaagaactggcgaaatacgacgctggcgttgctatcactctgtctgcaaccgtttctctgtgcgcaaacccgatctggcagttcggtactgaagcgcagaaagagaagttcctggttccgctggttgaaggtactaaactgggtgcattcggtctgactgaaccgaacgctggtactgacgcttctggtcagcagactatcgctaccaaaaacgacgacggtacttacactctgaacggttctaaaatcttcatcactaacggtggtgcagctgacatctacatcgttttcgcaatgactgacaagtctaaaggtaaccacggtatcactgcattcatcctggaagatggtactccgggcttcacttacggtaagaaagaagataaaatgggtatccacacttctcagactatggaactggtattccaggacgttaaagttccggcagaaaacatgctgggtgaagaaggtaaaggcttcaaaatcgcgatgatgactctggacggtggtcgtatcggtgttgctgctcaggcgctgggtatcgctgaagcggcactggctgacgcggtagaatactccaagcagcgtgtacagttcggtaagccgctgtgcaaattccagtctatctccttcaaactggctgatatgaagatgcagatcgaagcagctcgcaacctggtttacaaagcggcatgtaagaagcaggaaggtaagccgttcaccgttgatgctgctatcgctaaacgcgttgcttctgacgttgcgatgcgcgtaactactgaagctgttcagattttcggtggttacggttactctgaagaatacccggttgcgcgtcacatgcgtgacgctaaaatcactcagatttacgaaggtactaacgaagttcagctgatggttactggcggtgcgctgctgcgtgagctctaataagctt

SEQ ID NO: 105 - protein, 385 aa, Megasphaera elsdenii, Acyl-CoA dehydrogenase, short-chain specific;  EC=1.3.99.2 (Q06319)
MDFNLTDIQQDFLKLAHDFGEKKLAPTVTERDHKGIYDKELIDELLSLGITGAYFEEKYGGSGDDGGDVLSYILAVEELAKYDAGVAITLSATVSLCANPIWQFGTEAQKEKFLVPLVEGTKLGAFGLTEPNAGTDASGQQTIATKNDDGTYTLNGSKIFITNGGAADIYIVFAMTDKSKGNHGITAFILEDGTPGFTYGKKEDKMGIHTSQTMELVFQDVKVPAENMLGEEGKGFKIAMMTLDGGRIGVAAQALGIAEAALADAVEYSKQRVQFGKPLCKFQSISFKLADMKMQIEAARNLVYKAACKKQEGKPFTVDAAIAKRVASDVAMRVTTEAVQIFGGYGYSEEYPVARHMRDAKITQIYEGTNEVQLMVTGGALLRET

SEQ ID NO: 106 - DNA, 1421 bp, Artificial
  Acinetobacter sp. (strain ADP1), Acyl-CoA dehydrogenase; EC=1.3.99 (Q937T2)
ggtaccttttttgggctaacaggaggaattaaccatgatcaacaagatcatcaacgatatcgaaccgattctgaaatctatcccagacggttctaccatcatgacttctggcttcggtactaccggtcagccggaagcgctgctggaagcgctgatcgacttcgcaccgaaagagctgactatcatcaacaacaacgcttcttccggtccgaacggtctgactcagctgttcactgctggtctggttaagaaactgatctgctcctacccgaaatctatctcttccaccgttttcccggacctgtaccgcgctggtaagatcgaactggaactggttccgcagggtaacctggcttgccgtatccaggcagctggcgcgggtctgggtgcagtattcactccgactggttacggtactaagatcgctgaaggtaaagaaactcgtatcatcaacggtaaaaactacgttctggaatacccgctggaagctgactacgcattcatctacgctgacaaagctgaccgctggggtaacctgacttaccgtaaagcggcacgtaacttcggtccgatcatggcgaaagcagctaaaaccactattgctcaggttaaccagactgttgaactgggcgatctggacccggaatgcatcatcactccgggtatcttcgtacagcacgttgttcgtctgggtgacatcaaataattttttgggctaacaggaggaattaaccatgactattcagaagcgttctcgcgaagatatcgctatcatgatcgctaaagacatcccggacggttcttacgttaacctgggtatcggtctgccgactcacgttgctaaatatctgccgaaagacaaagaaatcttcctgcactctgaaaacggtgttctggcattcggtccgccgccagcagaaggtgaagaagatcaggacctggttaacgctggtaaagagctggtaactctgctgtctggtggttgcttcatgcaccacggtgactccttcgacatcatgcgtggtggtcacctggatatctgcgttatcggtgcattccaggttgcgctgaacggtgacctggctaactggcacaccggtaaagacgacgacgttccggcagtaggtggtgcaatggacctggctgttggtgcgaagcgtatcttcgtttacatggaacacaccaccaagaaaggtgaaccgaaaatcgttaagcacctgacttacccgatcaccggtgaacagtgcgtagaccgtatctacactgacctgtgcaccatcgaactgaaagacggtcaggcttacgttatcgaaatggttgacggtctggatttcgacactctgcaggcgctgactgaatgcccgctgatcgaccactgcacctactcttctctgattcagctcagataaggatccgagctc

SEQ ID NO: 107 - protein, 223 aa, Acinetobacter sp. (strain ADP1), Acyl-CoA dehydrogenase;  EC=1.3.99 (Q937T2)
MINKIINDIEPILKSIPDGSTIMTSGFGTTGQPEALLEALIDFAPKELTIINNNASSGPNGLTQLFTAGLVKKLICSYPKSISSTVFPDLYRAGKIELELVPQGNLACRIQAAGAGLGAVFTPTGYGTKIAEGKETRIINGKNYVLEYPLEADYAFIYADKADRWGNLTYRKAARNFGPIMAKAAKTTIAQVNQTVELGDLDPECIITPGIFVQHVVRLGDIK

SEQ ID NO: 108 - DNA, 1190 bp, Artificial
  Deinococcus radiodurans, Acyl-CoA dehydrogenase (Q9RVV0)
ggtaccggatccctaacaggaggaattaaccatggacttcaatctgccggacgatctgcgtgaagttcaggcaactatccgtgacttcatgctgactcgcgttgaagatcgcgctcaggaaatcgaacacaccaactccgtaccgccggaactgatcaaagaagcggcagacctgggtctgttcggtctgtctatcccggaagaatacggtggtgttggtctgtcctctctgggtcgttgcgcagtttacgaagcgatgggtcagggtcacatgggcttcggtggtatgatctccgcacacgcttctatcggtacttctggtctggttaaactgggtaacgaagagcagaagcagcgtttcctgccgcgtatggcggcaggcgaatgcatcgctggcttcgctatcactgaaccaagctccggttctgacgctggtaacatccgtactaaagctgttaagaaaggcgacgtttacgttctgaacggtactaagcactacatctccaacgctccgatcgctggtctgctgaccgttatcgctatcactgacccggcacagggttcccgtggtatgtccgcattcctggttgaaccgcagtctactccgggcgtatctatcggtaaaatcgacgaaaaaatgggtcagaaaggtgcgctgtctgcagaagttatcttcgaagatgctgaaatcccggctgctaaccttctcggtccggaaaaccgcggttaccgtgaagcgctgggtattctgactaacggtcgcgttggtatcgctgcacgttctactggcgcgatgcagcgtctgctggacctgtctgttgcacacgctcagactcgcgagcagttcggtaagccgatcgctgagttccaggcggtacagttcatgctggcagaaatggaagttgcgattcagacttctcgcgtactgtggcagaaagttgcatggatggttgaccagggtcaggacgttaagcgtatggcgtctgttgctaaataccacgcaactgaaatgctgtctcaggttgctgacaaagcggtacaggttgctggcggtatgggttacgttaaagacgctccgttcgaacgtttctaccgcgaccagcgtctgctgcgtatctacgaaggtacttctgaaatccagaaagttatcatcgctgctgaactgctgcgtcgcgagctctaataagctt

SEQ ID NO: 109 - protein, 383 aa, Deinococcus radiodurans, Acyl-CoA dehydrogenase (Q9RVV0)
MDFNLPDDLREVQATIRDFMLTRVEDRAQEIEHTNSVPPELIKEAADLGLFGLSIPEEYGGVGLSSLGRCAVYEAMGQGHMGFGGMISAHASIGTSGLVKLGNEEQKQRFLPRMAAGECIAGFAITEPSSGSDAGNIRTKAVKKGDVYVLNGTKHYISNAPIAGLLTVIAITDPAQGSRGMSAFLVEPQSTPGVSIGKIDEKMGQKGALSAEVIFEDAEIPAANLLGPENRGYREALGILTNGRVGIAARSTGAMQRLLDLSVAHAQTREQFGKPIAEFQAVQFMLAEMEVAIQTSRVLWQKVAWMVDQGQDVKRMASVAKYHATEMLSQVADKAVQVAGGMGYVKDAPFERFYRDQRLLRIYEGTSEIQKVIIAAELLRRET

SEQ ID NO: 110 - DNA, 1202 bp, Artificial
  Arabidopsis thaliana, Isovaleryl-CoA dehydrogenase, mitochondrial;  Short=IVD;  EC=1.3.99.10
ggtaccggatccctaacaggaggaattaaccatggcctcttctctgctgttcgacgacactcagctgcagttcaaagaatccgtttccaagttcgctcaggacaacatcgctccgcacgctgaacgtatcgacaaaactaactccttcccgaaagacgttaacctgtggaaactgatgggcgagttcaatctgcacggtatcactgcgccagaagaatacggtggtctgggtctgggttacctgtaccactgcatcgcgatggaagaaatctctcgcgcttctggttctgttgctctgtcttacggcgcacactctaacctgtgcatcaaccagctggtacgtaacggtactgctgcacagaaagagaagtatctgccgaaactgatctccggtgaacacgttggtgcactggcgatgtctgaaccgaacgctggttctgacgttgttggtatgaagtgcaaagcagaaaaagttgacggtggttacattctgaacggtaacaagatgtggtgcaccaacggtccgtctgctgaaactctggttgtttacgctaaaactgacaccaaagcgggttctaaaggtatcactgcattcatcatcgaaaaaggtatgaccggtttctccactgctcagaagctggacaagctgggtatgcgcggttctgacacttgcgaactggtattcgaaaactgcttcgtaccggaagaaaacatcctggataaagaaggtaaaggcgtttacgttctgatgtccggtctggatctggaacgtctggtactggcagctggtccgctgggtatcatgcaggcttgcctggataacgtactgccgtacatccgtcagcgtgaacagttcggtcgtccggttggcgagttccagttcatccagggtaaagttgctgacatgtacactgcgctgcagtcctcccgttcttacgtttactccgttgctcgcgactgcgacaacggtaaagttgatccgaaagactgcgcaggcactatcctgtgcgcagctgaacgtgcaactcaggttgcgctgcaggcgattcagtgcctgggtggtaacggttacatcaacgaatacgcaactggtcgtctgctgcgcgacgcgaagctgtacgaaatcggtgctggtacttctgaaatccgccgtatcgttatcggtcgtgaactgttcaaagaagaagagctctaataagctt

SEQ ID NO: 111 - protein, 387 aa, Arabidopsis thaliana, Isovaleryl-CoA dehydrogenase, mitochondrial;  Short=IVD;  EC=1.3.99.10
MASSLLFDDTQLQFKESVSKFAQDNIAPHAERIDKTNSFPKDVNLWKLMGEFNLHGITAPEEYGGLGLGYLYHCIAMEEISRASGSVALSYGAHSNLCINQLVRNGTAAQKEKYLPKLISGEHVGALAMSEPNAGSDVVGMKCKAEKVDGGYILNGNKMWCTNGPSAETLVVYAKTDTKAGSKGITAFIIEKGMTGFSTAQKLDKLGMRGSDTCELVFENCFVPEENILDKEGKGVYVLMSGLDLERLVLAAGPLGIMQACLDNVLPYIRQREQFGRPVGEFQFIQGKVADMYTALQSSRSYVYSVARDCDNGKVDPKDCAGTILCAAERATQVALQAIQCLGGNGYINEYATGRLLRDAKLYEIGAGTSEIRRIVIGRELFKEEET

SEQ ID NO: 112 - DNA, 1232 bp, Artificial
  Homo sapiens, Glutaryl-CoA dehydrogenase, mitochondrial; Short=GCD;  EC=1.3.99.7 (Q92947)
ggtaccggatccctaacaggaggaattaaccatgggtccggaatttgactggcaggacccgctggtactggaagagcagctgaccactgacgaaatcctgatccgtgacaccttccgtacttactgccaggaacgtctgatgccgcgcattctgctggctaaccgtaacgaagttttccaccgtgaaatcatctctgaaatgggtgaactgggtgttctgggtccgactatcaaaggttacggttgcgcaggcgtttcttccgttgcttacggtctgctggcgcgtgaactggaacgcgttgactccggttaccgttctgcaatgtccgttcagtcctctctggtaatgcacccaatctacgcttacggttctgaagagcagcgtcagaaatatctgccgcagctggcgaaaggtgaactgctgggttgcttcggtctgactgaaccgaactccggttctgacccgtcctctatggaaactcgcgcacactacaactcttctaacaagtcttacactctgaacggcaccaaaacctggatcactaactctccgatggctgacctgttcgttgtatgggctcgctgcgaagatggttgcatccgcggtttcctgctggaaaaaggtatgcgtggtctgtctgcaccgcgtatccagggtaagttctctctgcgcgcttctgcaactggtatgatcatcatggacggtgttgaagttccggaagaaaacgttctgccgggtgcatcttctctgggtggtccgttcggttgcctgaacaacgcgcgttacggtatcgcatggggcgtactgggtgcttctgagttctgcctgcacactgcacgtcagtacgcactggatcgcatgcagttcggtgttccgctggcgcgtaaccagctgattcagaagaaactggctgacatgctgactgaaatcactctgggtctgcacgcttgcctgcagctgggtcgtctgaaagaccaggacaaagctgcaccggaaatggtttctctgctgaagcgtaacaactgcggtaaagcgctggatatcgctcgccaggctcgcgacatgctgggtggtaacggtatctctgacgaataccacgttatccgtcacgcgatgaacctggaagctgttaacacctacgaaggtactcacgacatccacgcgctgatcctgggtcgtgctatcaccggtatccaggctttcactgcttctaaagagctctaataagctt

SEQ ID NO: 113 - protein, 397 aa, Homo sapiens, Glutaryl-CoA dehydrogenase, mitochondrial;  Short=GCD;  EC=1.3.99.7 (Q92947)
MGPEFDWQDPLVLEEQLTTDEILIRDTFRTYCQERLMPRILLANRNEVFHREIISEMGELGVLGPTIKGYGCAGVSSVAYGLLARELERVDSGYRSAMSVQSSLVMHPIYAYGSEEQRQKYLPQLAKGELLGCFGLTEPNSGSDPSSMETRAHYNSSNKSYTLNGTKTWITNSPMADLFVVWARCEDGCIRGFLLEKGMRGLSAPRIQGKFSLRASATGMIIMDGVEVPEENVLPGASSLGGPFGCLNNARYGIAWGVLGASEFCLHTARQYALDRMQFGVPLARNQLIQKKLADMLTEITLGLHACLQLGRLKDQDKAAPEMVSLLKRNNCGKALDIARQARDMLGGNGISDEYHVIRHAMNLEAVNTYEGTHDIHALILGRAITGIQAFTASKET

SEQ ID NO: 114 - DNA, 1784 bp, Artificial
  Homo sapiens, Electron transfer flavoprotein subunit alpha, mitochondrial (P13804)
ggtaccggatccctaacaggaggaattaatcatgaccactctggttatcgctgaacacgctaacgactctctggcaccaatcactctgaacaccatcactgcggcaactcgtctgggtggtgaagtttcctgcctggttgctggcaccaagtgcgacaaagttgctcaggacctgtgcaaagtagcgggtatcgcgaaagttctggtagcgcagcacgacgtttacaaaggtctgctgccggaagagctgactccgctgatcctggcaactcagaagcagttcaactacactcacatctgtgcgggtgcttctgcattcggtaaaaatctgctgccgcgcgttgctgcgaaactggaagttgcaccgatttctgacatcatcgctatcaagtctccggataccttcgtacgtactatctacgctggtaacgcactgtgcaccgttaagtgcgacgaaaaagttaaagtattctctgtacgtggtacttctttcgacgctgcagcaacttctggtggttctgcatcttctgaaaaagcatcttccacttctccggttgaaatctctgagtggctggatcagaaactgaccaagtctgaccgtccggaactgactggcgcgaaagttgttgtttctggtggtcgtggtctgaaatctggtgaaaacttcaaactgctgtacgacctggctgaccagctgcacgctgctgttggtgcttctcgcgctgctgttgatgctggcttcgtaccgaacgacatgcaagttggtcagactggtaaaatcgttgcaccggaactgtacatcgctgttggtatctccggtgcgattcagcacctggcgggtatgaaagactccaaaactatcgttgctatcaacaaagacccggaagcaccgatcttccaggttgctgactacggtatcgttgctgacctgttcaaagttgttccggaaatgactgaaatcctgaagaagaagtaataactagtctaacaggaggaattaaccatggctgaactgcgcgtactggttgctgttaagcgcgttatcgactacgcagttaaaatccgcgttaagccggaccgtactggcgttgttactgacggtgttaaacactctatgaacccgttctgcgaaatcgctgttgaagaagcggtacgtctgaaagagaagaaactggttaaagaagttatcgctgtttcctgcggtccggcacagtgccaggaaaccattcgtactgcactggcgatgggcgcagaccgcggtatccacgttgaagttccgccagctgaagcagaacgtctgggtccgctccaggttgctcgcgtactggcgaaactggctgaaaaagaaaaagttgacctggtactgctgggtaagcaggctatcgacgacgactgcaaccagactggtcagatgactgctggcttcctggactggccgcagggtactttcgcttctcaggtaactctggaaggtgacaaactgaaagttgaacgtgaaatcgacggtggtctggaaactctgcgtctgaaactgccggcagttgttactgctgatctgcgtctgaacgaaccgcgttacgcaactctgccgaacattatgaaagcgaagaagaagaaaatcgaagttatcaagccgggcgacctgggtgttgacctgacttctaaactgtctgttatctccgttgaagatccgccgcagcgtactgctggcgttaaagttgaaaccactgaggatctggtagcgaaactgaaagaaatcggtcgtatcgagctctaataagctt

SEQ ID NO: 115 - protein, 314 aa, Homo sapiens, Electron transfer flavoprotein subunit alpha, mitochondrial (P13804)
MTTLVIAEHANDSLAPITLNTITAATRLGGEVSCLVAGTKCDKVAQDLCKVAGIAKVLVAQHDVYKGLLPEELTPLILATQKQFNYTHICAGASAFGKNLLPRVAAKLEVAPISDIIAIKSPDTFVRTIYAGNALCTVKCDEKVKVFSVRGTSFDAAATSGGSASSEKASSTSPVEISEWLDQKLTKSDRPELTGAKVVVSGGRGLKSGENFKLLYDLADQLHAAVGASRAAVDAGFVPNDMQVGQTGKIVAPELYIAVGISGAIQHLAGMKDSKTIVAINKDPEAPIFQVADYGIVADLFKVVPEMTEILKKK

SEQ ID NO: 116 - protein, 255 aa, Homo sapiens, Electron transfer flavoprotein subunit beta (P38117); identical to SEQ ID NO: 92

SEQ ID NO: 117 - protein, 316 aa, Homo sapiens Acyl-coenzyme A thioesterase 8,     EC=3.1.2.27 (O14734)
MSSPQAPEDGQGCGDRGDPPGDLRSVLVTTVLNLEPLDEDLFRGRHYWVPAKRLFGGQIVGQALVAAAKSVSEDVHVHSLHCYFVRAGDPKLPVLYQVERTRTGSSFSVRSVKAVQHGKPIFICQASFQQAQPSPMQHQFSMPTVPPPEELLDCETLIDQYLRDPNLQKRYPLALNRIAAQEVPIEIKPVNPSPLSQLQRMEPKQMFWVRARGYIGEGDMKMHCCVAAYISDYAFLGTALLPHQWQHKVHFMVSLDHSMWFHAPFRADHWMLYECESPWAGGSRGLVHGRLWRQDGVLAVTCAQEGVIRVKPQVSE

SEQ ID NO: 118 - DNA, 931 bp, Artificial
  Hyphomonas neptunium Acyl-CoA thioesterase (Q0BZ30)
ggtaccttttttgggctaacaggaggaattaaccatggcgaaagacccggttggcgatctgctgactctgctggatctggaacgtctggaactggatctgttccgcggtcagtctccggacgaagaagaatctcagcgcgtattcggtggtcaggttatcgctcagtctctggttgctgcttaccgtactgtaccggacgaccgtctgtgccactctctgcactgctacttcatccgtccgggcgacccgtctgtaccaatcatctaccaggttgaccactctcgcgacggtggttctttcaccactcgtcgcgttgttgctatccagcacggtaagcagattttcaacctggcagcttctttccacgttgttgaagattcctggcaccaccagcacgaaatgccggaagttgacccgccagaatccgtaggtgaccgtatcgagtggcgtcgtaaattcgctgaacaggttccggaacgtcaccgcggtcacttcctgcgcgaccgtccggttgaaatgcgtgaaatcgacccgctggacccgctgaaaccggcaaaagcgtctgaccagcagaacctgtggttccgcgttgctcgtccgatcgacgaagcgccgtggctgcaccactgcctgatggcttacgcttctgacatggcgctgctgggtactggtaaccgtccgcacggtatctcctggatgaccggtgaactgatgtccgcatctctggatcacgcgatgtggttccacgcaccgactaaattcgacgagtggcacctgtactctatggactctccgtacgcaggcggtgcacgttctttcaaccgcggttctatctacgactccaccggtcgtctggttgcttctgttgctcaggaaggtctgatgcgtcgcgttgaacgtaagccgcgtaaaagctaaggatccgagctc

SEQ ID NO: 119 - protein, 294 aa, Hyphomonas neptunium Acyl-CoA thioesterase (Q0BZ30)
MAKDPVGDLLTLLDLERLELDLFRGQSPDEEESQRVFGGQVIAQSLVAAYRTVPDDRLCHSLHCYFIRPGDPSVPIIYQVDHSRDGGSFTTRRVVAIQHGKQIFNLAASFHVVEDSWHHQHEMPEVDPPESVGDRIEWRRKFAEQVPERHRGHFLRDRPVEMREIDPLDPLKPAKASDQQNLWFRVARPIDEAPWLHHCLMAYASDMALLGTGNRPHGISWMTGELMSASLDHAMWFHAPTKFDEWHLYSMDSPYAGGARSFNRGSIYDSTGRLVASVAQEGLMRRVERKPRKS

SEQ ID NO: 120 - DNA, 1421 bp, Artificial; identical to SEQ ID NO: 106
  Acinetobacter sp. (strain ADP1), Acyl-CoA-transferase subunit A (EC=2.8.3.6) (Q937T0)

SEQ ID NO: 121 - protein, 223 aa, Acinetobacter sp. (strain ADP1), Acyl-CoA-transferase subunit A (EC=2.8.3.6) (Q937T0); identical to SEQ ID NO: 107

SEQ ID NO: 122 - protein, 224 aa, Acinetobacter sp. (strain ADP1) Acyl-CoA-transferase subunit B (EC 2.8.3.6)  (Q937S9)
MTIQKRSREDIAIMIAKDIPDGSYVNLGIGLPTHVAKYLPKDKEIFLHSENGVLAFGPPPAEGEEDQDLVNAGKELVTLLSGGCFMHHGDSFDIMRGGHLDICVIGAFQVALNGDLANWHTGKDDDVPAVGGAMDLAVGAKRIFVYMEHTTKKGEPKIVKHLTYPITGEQCVDRIYTDLCTIELKDGQAYVIEMVDGLDFDTLQALTECPLIDHCTYSSLIQLR

SEQ ID NO: 123 - protein, 437 aa, Clostridium kluyveri (strain ATCC 8527) acetate CoA-transferase activity (A5N390)
MVFKNWQDLYKSKIVSADEAVSKVSCGDSIILGNACGASLTLLDALAANKEKYKSVKIHNLILNYKNDIYTDPESEKYIHGNTFFVSGGTKEAVNCNRTDYTPCFFYEIPKLLKQKYINADVAFIQVSKPDSHGYCSFGVSTDYSQAMVQSAKLIIAEVNDQMPRVLGDNFIHISDMDYIVESSRPILELTPPKIGEVEKTIGKYCASLVEDGSTLQLGIGAIPDAVLLFLKDKKDLGIHSEMISDGVVELVEAGVITNKKKSLHPGKIIITFLMGTKKLYDFINDNPMVEGYPVDYVNDPKVIMQNSKMVCINSCVEVDFTGQVCAESVGFKQISGVGGQVDYMRGASMADGGKSILAIPSTAAGGKISRIVPILTEGAGVTTSRYDVQYVVTEYGIALLKGKSIRERAKELIKIAHPKFREELTAQFEKRFSCKL

SEQ ID NO: 124 - protein, 538 aa, Clostridium kluyveri (strain ATCC 8527) Succinyl-CoA:coenzyme A transferase (P38946)
MSKGIKNSQLKKKNVKASNVAEKIEEKVEKTDKVVEKAAEVTEKRIRNLKLQEKVVTADVAADMIENGMIVAISGFTPSGYPKEVPKALTKKVNALEEEFKVTLYTGSSTGADIDGEWAKAGIIERRIPYQTNSDMRKKINDGSIKYADMHLSHMAQYINYSVIPKVDIAIIEAVAITEEGDIIPSTGIGNTATFVENADKVIVEINEAQPLELEGMADIYTLKNPPRREPIPIVNAGNRIGTTYVTCGSEKICAIVMTNTQDKTRPLTEVSPVSQAISDNLIGFLNKEVEEGKLPKNLLPIQSGVGSVANAVLAGLCESNFKNLSCYTEVIQDSMLKLIKCGKADVVSGTSISPSPEMLPEFIKDINFFREKIVLRPQEISNNPEIARRIGVISINTALEVDIYGNVNSTHVMGSKMMNGIGGSGDFARNAYLTIFTTESIAKKGDISSIVPMVSHVDHTEHDVMVIVTEQGVADLRGLSPREKAVAIIENCVHPDYKDMLMEYFEEACKSSGGNTPHNLEKALSWHTKFIKTGSMK

SEQ ID NO: 125 - protein, 232 aa, Pseudomonas fluorescens (strain Pf-5 / ATCC BAA-477) 3-oxoacid CoA-transferase subunit A family enzyme (Q4KEA3)
MAGFDKRVASYEEALEGLQDGMTVIAGGFGLCGIPENLIAEIKRRGTRDLTVVSNNCGVDGFGLGVLLEDRQISKVIASYVGENALFEKQLLSGEIEVVLTPQGTLAEKMRAGGAGIPAFFTATGVGTPVADGKETREFKGRTYLMEESITGDFAIVKGWKADHFGNVVYRHTAQNFNPLAATAGKITVVEVEEIVEPGELDPTQIHTPGIYVDRVICGTFEKRIEQRTVRK

SEQ ID NO: 126 - protein, 219 aa, Pseudomonas fluorescens (strain Pf-5 / ATCC BAA-477) 3-oxoacid CoA-transferase subunit B family enzyme (Q4KEA4)
MALTREQMAQRVARELQDGFYVNLGIGIPTLVANYIPDGMEVMLQSENGLLGMGAFPTEDEVDADMINAGKQTVTARIGASIFSSAESFAMIRGGHIDLTVLGAFEVDVQGNIASWMIPGKLVKGMGGAMDLVAGAENIIVTMTHASKDGESKLLSRCSLPLTGAQCIKRVLTDLAYLEIENGAFILKERAPGVSVEEIVSKTAGKLIVPDHVPEMQFA

SEQ ID NO: 127 - protein, 477 aa, Acinetobacter sp. NCIMB9871 6-oxohexanoate dehydrogenase (Q9R2F4)
MNYPNIPLYINGEFLDHTNRDVKEVFNPVNHECIGLMACASQADLDYALESSQQAFLRWKKTSPITRSEILRTFAKLAREKAAEIGRNITLDQGKPLKEAIAEVTVCAEHAEWHAEECRRIYGRVIPPRNPNVQQLVVREPLGVCLAFSPWNFPFNQAIRKISAAIAAGCTIIVKGSGDTPSAVYAIAQLFHEAGLPNGVLNVIWGDSNFISDYMIKSPIIQKISFTGSTPVGKKLASQASLYMKPCTMELGGHAPVIVCDDADIDAAVEHLVGYKFRNAGQVCVSPTRFYVQEGIYKEFSEKVVLRAKQIKVGCGLDASSDMGPLAQARRMHAMQQIVEDAVHKGSKLLLGGNKISDKGNFFEPTVLGDLCNDTQFMNDEPFGPIIGLIPFDTIDHVLEEANRLPFGLASYAFTTSSKNAHQISYGLEAGMVSINHMGLALAETPFGGIKDSGFGSEGGIETFDGYLRTKFITQLN

SEQ ID NO: 128 - protein, 473 aa, Brucella melitensis  6-oxohexanoate dehydrogenase (Q8YDF1)
MRIGKMEMQTRYPDVKLFIDGTWRDGSRGETIEIFNPATDEVIGHIARATTADLDDALAAVDRGFEAWSKVSAFDRYKIMRRAADIFRSRGEEVARLLTMEQGKPLAEARIEAAAACDLIDWFAEEARRSYGRIVPPRQAYVMQAEVKEPVGPVAAFTPWNFPINQAVRKISAALAAGCSILLKAAEDTPAAPAELVRAFAEAGLPDGAINLVYGDPAEISAYLIPHPVIRKVSFTGSTQVGKQLAALAGLHMKRVTMELGGHAPVIIAADADVEQAIKVVSGSKFRNAGQVCISPTRFLIENSVYDQVVEGMAAYATSLKVGDGLEAGTTMGPLVNAKRVNAMERLVQDAREHKARVVTGGERIGNRGNFFEPTILADVPRDAAIMNEEPFGPVALLNRFDALDEALSEANRLNYGLAAYAFTGSSAKAARISSTVRSGMITINQLRSGPAGSALRRDQRFRLWNGRRCRRA

SEQ ID NO: 129 - DNA, 1371 bp, Artificial
  Pseudomonas aeruginosa (gi 9946143)
atgaacagccaaatcaccaacgccaagacccgtgagtggcaggcgttgagccgcgaccaccatctgccgccgttcaccgactacaagcagttgaacgagaagggcgcgcggatcatcaccaaggccgaaggcgtctatatctgggacagcgagggcaacaagatcctcgatgcgatggccggcctctggtgcgtcaacgtcggctacggccgcgaggagctggtccaggccgccacccggcagatgcgcgagttgccgttctacaacctgttcttccagaccgcccacccgccggtggtcgagctggccaaggcgatcgccgacgtcgctccggaaggcatgaaccacgtgttcttcaccggctccggctccgaggccaacgacaccgtgctgcgtatggtccgccactattgggcgaccaagggccagccgcagaagaaagtggtgatcggccgctggaacggctaccacggctccaccgtcgccggcgtcagcctgggcggcatgaaggcgttgcatgagcagggtgatttccccatcccgggcatcgtccacatcgcccagccctactggtacggcgagggcggcgacatgtcgccggacgagttcggcgtctgggccgccgagcagttggagaagaagattctcgaagtgggcgaggaaaacgtcgccgccttcatcgccgagccgatccagggcgccggcggcgtgatcgtcccgccggacacctactggccgaagatccgcgagatcctcgccaagtacgacatcctgttcatcgccgacgaagtgatctgcggcttcggccgtaccggcgagtggttcggcagccagtactacggcaacgccccggacctgatgccgatcgccaagggcctcacctccggctacatccccatgggcggggtggtggtgcgcgacgagatcgtcgaagtgctcaaccagggcggcgagttctaccacggcttcacctattccggtcacccggtggcggccgccgtggccctggagaacatccgcatcctgcgcgaagagaagatcatcgagaaggtgaaggcggaaacggcaccgtatttgcagaaacgctggcaggagctggccgaccacccgttggtgggcgaagcgcgcggggtcggcatggtcgccgccctggagctggtcaagaacaagaagacccgcgagcgtttcaccgacaagggcgtcgggatgctgtgccgggaacattgtttccgcaacggtttgatcatgcgcgcggtgggcgacactatgattatctcgccgccgctggtgatcgatccgtcgcagatcgatgagttgatcaccctggcgcgcaagtgcctcgatcagaccgccgccgccgtcctggcttga

SEQ ID NO: 130 - protein, 456 aa, Pseudomonas aeruginosa (gi 9946143); identical to SEQ ID NO: 84

SEQ ID NO: 131 - DNA, 70 bp, Artificial
  primer
ggggacaagtttgtacaaaaaagcaggctaggaggaattaaccatgaacagccaaatcaccaacgccaag

SEQ ID NO: 132 - DNA, 49 bp, Artificial
  primer
ggggaccactttgtacaagaaagctgggttcaagccaggacggcggcgg

SEQ ID NO: 133 - DNA, 1353 bp, Artificial
  Bacillus subtilis aminotransferase gene (gi16077991)
atggagatgatggggatggaaaacattcagcaaaatcagggattaaagcaaaaagatgagcaatttgtgtggcatgccatgaagggagcgcatcaagcggacagcctgatagcccagaaggccgaaggggcctgggtaaccgacacagacggacgccgctatttggatgcgatgtccggtttgtggtgcgtcaacattggttacggcagaaaggagcttgcggaggctgcctatgagcaactaaaggagctgccttactacccgttaacgcaaagtcacgcacccgcaattcaactggcggaaaagctgaatgaatggcttggcggcgattatgttatttttttttccaacagcggatcggaagcaaacgaaactgcttttaaaattgcccgccagtaccatctgcaaaacggcgaccacagccgttataaattcatctcaagatatcgggcataccacggcaatacattgggagcgctctcagctaccggacaggcgcagcggaaatataaatacgagcctttgagccaagggttcctgcatgcagctccgccagatatataccggaatcctgatgatgcagacacgcttgaaagcgcaaatgaaatcgaccgcatcatgacatgggaattaagcgaaacgattgccggggtcattatggagcccatcattacaggcggaggcatcctaatgccgccggacggatatatgaagaaggtggaggacatttgccggcgccacggagcccttttgatttgcgatgaagtgatctgcgggtttggacggacaggtgagccgttcgggtttatgcactacggtgtgaagcctgatatcattacgatggcaaagggaatcacaagcgcgtatctgccattgtcagcgactgctgtgaaacgggacattttcgaagcgtatcagggggaagctccttatgaccgtttccgccacgtgaacacgttcggcggaagcccggctgcctgtgctttggcgttgaaaaacctgcaaattatggaggacgaacagctgattcagcgatcccgtgatcttggagcaaagcttttaggtgagcttcaagctctgagagaacacccggcagtcggggatgttagaggaaaagggctgctgatcggaatcgaactcgtcaaagacaaattgactaaagagccggctgatgccgccaaagtaaaccaagtggttgcggcgtgcaaagaaaaagggctgatcatcggcaaaaacggcgatacagtcgccggctacaacaatgtcatccacgttgcgccgccattttgcctgacagaagaggacctttcctttatcgtgaaaacggtgaaagaaagctttcaaacgatataa

SEQ ID NO: 134 - protein, 450 aa, amino acid sequence of B. subtilis aminotransferase (gi16077991)
MEMMGMENIQQNQGLKQKDEQFVWHAMKGAHQADSLIAQKAEGAWVTDTDGRRYLDAMSGLWCVNIGYGRKELAEAAYEQLKELPYYPLTQSHAPAIQLAEKLNEWLGGDYVIFFSNSGSEANETAFKIARQYHLQNGDHSRYKFISRYRAYHGNTLGALSATGQAQRKYKYEPLSQGFLHAAPPDIYRNPDDADTLESANEIDRIMTWELSETIAGVIMEPIITGGGILMPPDGYMKKVEDICRRHGALLICDEVICGFGRTGEPFGFMHYGVKPDIITMAKGITSAYLPLSATAVKRDIFEAYQGEAPYDRFRHVNTFGGSPAACALALKNLQIMEDEQLIQRSRDLGAKLLGELQALREHPAVGDVRGKGLLIGIELVKDKLTKEPADAAKVNQVVAACKEKGLIIGKNGDTVAGYNNVIHVAPPFCLTEEDLSFIVKTVKESFQTI

SEQ ID NO: 135 - DNA, 1407 bp, Artificial
  Pseudomonas aeruginosa aminotransferase gene (seq ID gi9951072)
atgaacgcaagactgcacgccacgtcccccctcggcgacgccgacctggtccgtgccgaccaggcccactacatgcacggctaccacgtgttcgacgaccaccgcgtcaacggctcgctgaacatcgccgccggcgacggcgcctatatctacgacaccgccggcaaccgctacctcgacgcggtgggcggcatgtggtgcaccaacatcggcctggggcgcgaggaaatggctcgcaccgtggccgagcagacccgcctgctggcctattccaatcccttctgcgacatggccaacccgcgcgccatcgaactctgccgcaagctcgccgagctggcccccggcgacctcgaccacgtgttcctcaccaccggcggttccaccgccgtggacaccgcgatccgcctcatgcactactaccagaactgccgcggcaagcgcgccaagaagcacgtcatcacgcggatcaacgcctaccacggctcgaccttcctcggcatgtcgctgggcggcaagagcgccgaccggccggccgagttcgacttcctcgacgagcgcatccaccacctcgcctgtccctattactaccgcgctccggaagggctgggcgaagccgagttcctcgatggcctggtggacgagttcgaacgcaagatcctcgaactgggcgccgaccgggtgggggcgttcatctccgagccggtgttcggctccggcggcgtgatcgtcccgcccgcgggctaccacaggcggatgtgggagctgtgccagcgctacgacgtgctgtacatctccgacgaagtggtgacctccttcggccgcctcggccacttcttcgccagccaggcggtgttcggcgtacagccggacatcatcctcaccgccaagggcctcacctccggctaccagccgctgggcgcgtgcatcttctcccggcgcatctgggaggtgatcgccgagccggacaagggccgctgcttcagccatggtttcacctactccggccacccggtggcctgcgcggcggcgctgaagaacatcgagatcatcgagcgcgagggcttgctcgcccacgccgacgaggtcggccgctacttcgaggagcgcctgcaaagcctccgcgacctgcccatcgtcggcgacgtgcgcgggatgcgcttcatggcctgtgtcgagttcgtcgccgacaaggcgagcaaggcgctgtttccggaaagcctgaacatcggcgagtgggtccacctgcgggcgcagaagcgcggcctgctggttcgtccgatcgtccacctgaacgtgatgtcgccgccgctgatcctcacccgcgaacaggtcgataccgtggtccgggtgctgcgcgagagcatcgaggaaaccgtggaggatcttgtccgcgccggtcaccggtaa

SEQ ID NO: 136 - protein, 468 aa, amino acid sequence of Pseudomonas aeruginosa  aminotransferase (seq ID gi9951072)
MNARLHATSPLGDADLVRADQAHYMHGYHVFDDHRVNGSLNIAAGDGAYIYDTAGNRYLDAVGGMWCTNIGLGREEMARTVAEQTRLLAYSNPFCDMANPRAIELCRKLAELAPGDLDHVFLTTGGSTAVDTAIRLMHYYQNCRGKRAKKHVITRINAYHGSTFLGMSLGGKSADRPAEFDFLDERIHHLACPYYYRAPEGLGEAEFLDGLVDEFERKILELGADRVGAFISEPVFGSGGVIVPPAGYHRRMWELCQRYDVLYISDEVVTSFGRLGHFFASQAVFGVQPDIILTAKGLTSGYQPLGACIFSRRIWEVIAEPDKGRCFSHGFTYSGHPVACAAALKNIEIIEREGLLAHADEVGRYFEERLQSLRDLPIVGDVRGMRFMACVEFVADKASKALFPESLNIGEWVHLRAQKRGLLVRPIVHLNVMSPPLILTREQVDTVVRVLRESIEETVEDLVRAGHR

SEQ ID NO: 137 - DNA, 1335 bp, Artificial
  Pseudomonas aeruginosa aminotransferase gene (seq ID gi9951630)
atgacaatgaatgacgagccgcagtcgagcagcctcgacaacttctggatgcccttcaccgccaaccgccagttcaaggcgcggccgcgcctgctggaaagcgccgaaggcatccactatatcgcccagggcgggcgccgcatcctcgacggcaccgccggcctctggtgctgcaatgccggccacggccggcgcgagatcagcgaagcggtggcccggcagatcgccaccctcgactacgccccgccgttccagatgggtcacccgctgccgttcgaactcgccgcgcggctgacggaaatcgccccgccgagcctgaacaaagtattcttcaccaactccggctcggaatcggcggacaccgcgctgaagatcgcccttgcctaccagcgcgccatcggccagggcacccgcacccgcctgatcggccgcgaactgggctaccacggggtcggcttcggcggcctgtcggtaggcggtatggtcaacaaccgcaaggccttctccgccaacctgctgccgggggtcgaccacctgccgcacaccctggacgtcgcccgcaacgccttcaccgtcggcctgcccgagcatggcgtggaaaaggccgaggagctggaacgcctggtgaccctgcacggcgccgagaatatcgccgcggtgatcgtcgagccgatgtccggctcggccggcgtggtgctgccgcccaagggctaccttcagcggctgcgcgagataacccgcaagcatggcatcctgctgatcttcgacgaagtgatcaccggtttcggccgcgtcggcgaagccttcgccgcgcagcgctggggcgtcgtcccggacctgctgacctgcgccaaggggctgaccaacggcagcatcccgatgggcgccgtattcgtcgacgagaagatccatgctgccttcatgcaaggcccgcagggcgccatcgagttcttccacggctatacctattccggccatccggtagcctgcgccgccgccctggcgaccctggacatctaccgtcgcgacgacctgttccagcgggccgtcgaactggaaggctactggcaggacgcgctgttcagcctgcgcgacctgcccaacgtggtcgacatccgcgccgtaggcctggtcggcggcgtgcaactggcgccgcacgcggacggccccggcaagcgcggctacgacgtcttcgagcgctgcttctgggagcacgacctgatggtccgggtgaccggcgacatcatcgccatgtcgccgccgctgatcatcgacaagccccacatcgaccagatcgtcgagcgcctggcccaggccatccgcgccagcgtctga

SEQ ID NO: 138 - protein, 444 aa, amino acid sequence of Pseudomonas aeruginosa  aminotransferase (seq ID gi9951630)
MTMNDEPQSSSLDNFWMPFTANRQFKARPRLLESAEGIHYIAQGGRRILDGTAGLWCCNAGHGRREISEAVARQIATLDYAPPFQMGHPLPFELAARLTEIAPPSLNKVFFTNSGSESADTALKIALAYQRAIGQGTRTRLIGRELGYHGVGFGGLSVGGMVNNRKAFSANLLPGVDHLPHTLDVARNAFTVGLPEHGVEKAEELERLVTLHGAENIAAVIVEPMSGSAGVVLPPKGYLQRLREITRKHGILLIFDEVITGFGRVGEAFAAQRWGVVPDLLTCAKGLTNGSIPMGAVFVDEKIHAAFMQGPQGAIEFFHGYTYSGHPVACAAALATLDIYRRDDLFQRAVELEGYWQDALFSLRDLPNVVDIRAVGLVGGVQLAPHADGPGKRGYDVFERCFWEHDLMVRVTGDIIAMSPPLIIDKPHIDQIVERLAQAIRASV

SEQ ID NO: 139 - protein, 467 aa, Escherichia coli (strain K12) Ethanolamine utilization protein eutE (P77445)
MNQQDIEQVVKAVLLKMQSSDTPSAAVHEMGVFASLDDAVAAAKVAQQGLKSVAMRQLAIAAIREAGEKHARDLAELAVSETGMGRVEDKFAKNVAQARGTPGVECLSPQVLTGDNGLTLIENAPWGVVASVTPSTNPAATVINNAISLIAAGNSVIFAPHPAAKKVSQRAITLLNQAIVAAGGPENLLVTVANPDIETAQRLFKFPGIGLLVVTGGEAVVEAARKHTNKRLIAAGAGNPPVVVDETADLARAAQSIVKGASFDNNIICADEKVLIVVDSVADELMRLMEGQHAVKLTAEQAQQLQPVLLKNIDERGKGTVSRDWVGRDAGKIAAAIGLKVPQETRLLFVETTAEHPFAVTELMMPVLPVVRVANVADAIALAVKLEGGCHHTAAMHSRNIENMNQMANAIDTSIFVKNGPCIAGLGLGGEGWTTMTITTPTGEGVTSARTFVRLRRCVLVDAFRIV

SEQ ID NO: 140 - protein, 532 aa, Clostridium tetani  Alcohol dehydrogenase (Q894U3)
MEKYDKDLYSIQQARNLARLGKVAANKIANYTEEQIDKILRNMVRVAEENAVSLAQMAVEETGFGKVEDKTYKNHLAATILYDSIKDMKTIGVISEDKVNKMIEIAEPVGLIMGIVPSTNPTSTAIFKSIIAIKSRNAIVFSPHPAAAKCTIRAVELMRDAAIEAGAPEDIIASLTNLTMEATNELMKNENVSLIIATGGPGMVKAAYSSGKPAIGVGAGNSPAYIERTANVEKAIRDIISSKSFDYGTICASEQSIICEECNHDAVVEELKKQGGYFMTAEETEKVCKLLFKNGHTMNAKFVGRSPQVIANAAGFTVSEDIKVLIGKQNGVGNGNPLSFEKLTTVLAFYTVKDWHEACELSIELLQNGIGHTMSIHTQNDDIVMEFAKKPASRILVNTGGSQGGTGASTGLKPAFTLGCGTWGGSSVSENVTPEHLINKKRVAYGLKDCATLVQNDPTFNCIKTASNCRGVKNQFMNMSPAQIAAAAEVLNKCNDYAKNTGCSNESKEKDANNEELLSLVNQIVAAMKGAN

SEQ ID NO: 141 - protein, 297 aa, Burkholderia thailandensis (strain E264 / ATCC 700388 )  Acetaldehyde dehydrogenase (Q2T7T0)
MKNKSSRTRVAILGSGSIGLDLMFKVKASEHFDLKFVVGRHANSDGLKLARSCNVETSSDGLDFLKENEDAYDLVFDATSAAAHKVNNGFFSGAGKFVIDLTPAKLGRLCVPCINLDDIGAEQNVNLITCGGQASLPLAYALKQAVDEIEYLEVVSAIASRSAGIATRENIDEYMTTTEYALAQFSGAKKTKAILNINPAEPGVRMQTTLYAHARYRDFDRVRACVAEMVEKVREYVPGYRLVVEPIESQGRITISLTVRGRGDYLPEYAGNLDIINCAALAVASHRHATARLGATQ

SEQ ID NO: 142 - protein, 316 aa, Pseudomonas putida  Acylating aldehyde dehydrogenase (Q9EVJ2)
MTRKVKAAIIGSGNIGTDLMIKILRHGQHIEMGAMVGIDPASDGLARAQRMGVAITHEGVEGLTRLPVFNEIDVVFDATSAGAHVKNEALLRERKPGLRMIDLTPAAIGPYCIPVVNGDDHLDATNVNMVTCGGQATIPMVAAVSRVAKVHYAEIIASISSKSAGPGTRANIDEFTETTSKAIEVVGGAAKGKAIIVLNPAEPPLMMRDTVYTLSDFADIDQIEESVQRMADAVQAYVPGYRLKQRVQFDRIEADCPIRIPGVGDRMNGLKTSIFLEVEGAAHYLPAYAGNLDIMTSAALRTAEKLAERLLASLVA

SEQ ID NO: 143 - protein, 539 aa, Burkholderia mallei  Acetaldehyde dehydrogenase (Acetylating) (A5XRR2)
MHRGAACWHGFGVTNGVAHVARRITDTDMRGATMNHADMQHLNIEFPYRKQYGNFIGGEWVAPVGGEYFDNVSPVTGRPFTAIPRSREADIELALDAAHAAKAGWAAKGAAERANVLLRIADRMEANLTRLAVAETIDNGKPLRETTAADVPLAIDHFRYFAGCIRAQEGSIADIGGDMVAYHFHEPLGVVGQIIPWNFPLLMAAWKLAPALAAGNCVVLKPAEQTPASILVFAELIQDLLPPGVLNIVNGFGLEAGKPLASSKRIAKIAFTGETSTGRLIMQYASENLIPVTLELGGKSPNIFFADVMDRDDSYFDKALEGFAMFALNQGEVCTCPSRALVEESIYDRFIERALKRVEAIKQGHPLDSQTMIGAQASAEQLEKILSYIDIGRGEGAQCLTGGERNVLGGELAEGYYVKPTVFRGHNKMRIFQEEIFGPVLAVTTFKTEEEALEIANDTLYGLGAGVWTRDGNRAYRFGRGIQAGRVWTNCYHAYPAHAAFGGYKQSGIGRETHKMMLDHYQQTKNLLVSYSEKPLGFF

SEQ ID NO: 144 - protein, 464 aa, Salmonella typhimurium Propanediol utilization CoA-dependent propionaldehyde dehydrogenase (Q9XDN1)
MNTSELETLIRTILSEQLTTPAQTPVQPQGKGIFQSVSEAIDAAHQAFLRYQQCPLKTRSAIISAMRQELTPLLAPLAEESANETGMGNKEDKFLKNKAALDNTPGVEDLTTTALTGDGGMVLFEYSPFGVIGSVAPSTNPTETIINNSISMLAAGNSIYFSPHPGAKKVSLKLISLIEEIAFRCCGIRNLVVTVAEPTFEATQQMMAHPRIAVLAITGGPGIVAMGMKSGKKVIGAGAGNPPCIVDETADLVKAAEDIINGASFDYNLPCIAEKSLIVVESVAERLVQQMQTFGALLLSPADTDKLRAVCLPEGQANKKLVGKSPSAMLEAAGIAVPAKAPRLLIALVNADDPWVTSEQLMPMLPVVKVSDFDSALALALKVEEGLHHTAIMHSQNVSRLNLAARTLQTSIFVKNGPSYAGIGVGGEGFTTFTIATPTGEGTTSARTFARSRRCVLTNGFSIR

SEQ ID NO: 145 - protein, 315 aa, Rhodococcus sp. (strain RHA1) Acetaldehyde dehydrogenase (Q0SJD4)
MSTTKVAVIGSGNIGTDLVIKLEQVAKNVEIAVLVGIDPASDGLARARRLGISTVDTGVQGLIEHPEFDDIEIIFDSTSAKAHLTNAEALRPYGKHLIDLTPAAIGPYVVPAVNLDQHLGAPDVNMVTCGGQATIPIVAAISKVTDVHYAEIVASIASKSAGPGTRANIDEFTETTAKAIEEVGGAAHGKAIIVLNPADPPLIMRDTVLALVSNPDQDAIRQSITDMVATVAAYVPGYRLKQDVQFTELGGADTVATLTGGADIGSPVWKVSVFLEVEGAAHYLPAYAGNLDIMTSAALQVAEKLAERTALEIAR

SEQ ID NO: 146 - protein, 468 aa, Clostridium beijerinckii Coenzyme A acylating aldehyde dehydrogenase (Q9X681)
MNKDTLIPTTKDLKLKTNVENINLKNYKDNSSCFGVFENVENAINSAVHAQKILSLHYTKEQREKIITEIRKAALENKEVLATMILEETHMGRYEDKILKHELVAKYTPGTEDLTTTAWSGDNGLTVVEMSPYGVIGAITPSTNPTETVICNSIGMIAAGNAVVFNGHPGAKKCVAFAIEMINKAIISCGGPENLVTTIKNPTMESLDAIIKHPLIKLLCGTGGPGMVKTLLNSGKKAIGAGAGNPPVIVDDTADIEKAGKSIIEGCSFDNNLPCIAEKEVFVFENVADDLISNMLKNNAVIINEDQVSKLIDLVLQKNNETQEYFINKKWVGKDAKLFSDEIDVESPSNIKCIVCEVNANHPFVMTELMMPILPIVRVKDIDEAVKYTKIAEQNRKHSAYIYSKNIDNLNRFEREIDTTIFVKNAKSFAGVGYEAEGFTTFTIAGSTGEGITSARNFTRQRRCVLAG

SEQ ID NO: 147 - protein, 475 aa, Bacillus thuringiensis serovar israelensis Alcohol dehydrogenase / Acetaldehyde dehydrogenase (Acetylating) (Q3EZP1)
MTNKTDEKEVQAMVNVVIKDENDVQEVVNTLVENGKEALKALESYTQEQVDHIVHEMALSGLDQHMPLAKMAVEETGRGVYEDKCTKNIFATEYIWHSIKKDKTVGIIHEDPHEEVIEIAEPVGVVAGVTPVTNPTSTTMFKAIIAMKTRNPIIFAFHPSAQQCSVAAAKILRDAAIRAGAPENCIQWIEKPSVEATKRLMNHEGVALVLATGGAGMVKSAYSTGKPALGVGPGNVPCYLEKSAHVKRAVNDLILSKTFDNGMICASEQAIIVDKEIYNGVKKEMQDNNCYFVTEEERIKLEKLVINENTCAVNSDIVGKSAHYIASLVSIKVPEDTKILVAEIKGVGAEYPLSREKLSPVLACIKANSQEEGFKYCEEMLNLGGLGHSAVIHSTNKEVQKQFGLRMKACRLIVNSPSAQGGIGDIYNAFIPSLTLGCGSYGKNSVSQNVTATHIINVKRLANSPDNMRGFTITT

SEQ ID NO: 148 - protein, 467 aa, marine gamma proteobacterium Aldehyde dehydrogenase (NAD) family protein (B7RWJ8)
MSEAQSPAQEVAEMMSRARAAQAQIADYTQEQVDELITAMVYAVAREDRSEEIARFTVEETQLGNYEGKYLKIHRKTRATLMDIIDDKSVGVIEELPERNIVKIAKPVGVIGALSPSTNPEATPVIKAISAVKGRNAIIVAPHPRAKLTNKKICDYMREALELCGAPADLVQSIDVPSLDKTNELMAQCDRVLATGGEAMVTAAYSSGTPALGVGVGNAVITVDDTADLDEAAEKIRISKTLDLAASCSSDNSVLVFESVYNELLEKLKHEGGFVIEGDDKAKLQSVIWEDDHLNAKIVAQHAQTICGQAGIDLPEGKSFLIVPETGAGADHPFSGEKLTVTMALYKVKDIDEAIEMTNKIQAYQGQGHSCGIYSYNDDNVLKLADATRTSRVMVNQPQAASNSGNLWNGMRQTFSLGCGSWGGNSINHNITWRDLINETWVSKPLATTKTIPSDEELFGAVMAKFS